European Patent Application EP 4 332 224 A2, published March 6, 2024. Title: RNA AND DNA BASE EDITING VIA ENGINEERED ADAR RECRUITMENT. Applicant: THE REGENTS OF THE UNIVERSITY OF CALIFORNIA. Application EP. The sequence listing filed with the application follows.

SEQUENCE LISTING (255 sequences)

SEQ ID NO: 1 - DNA, 323 bp, synthetic construct
  misc_feature 1..323: note = Description of Artificial Sequence: Synthetic polynucleotide
  modified_base 117..146: mod_base = OTHER; note = a, c, t, g, unknown or other
  modified_base 148..176: mod_base = OTHER; note = a, c, t, g, unknown or other
  source 1..323: mol_type = other DNA
ggccgggcgcggtggctcacgcctgtaatcccagcactttgggaggccgaggcggggagattgcttgagcccaggagttcgagaccagcctgggcaacatagcgagaccccgtctcnnnnnnnnnnnnnnnnnnnnnnnnnnnnnncnnnnnnnnnnnnnnnnnnnnnnnnnnnnnagccgggcgtggtggcgcgcgcctgtagtcccagctactcgggaggctgaggcaggaggatcgcttgagcccaggagttcgaggctgcagtgagctatgatcgcgccactgcactccagcctgggcgacagagcgagaccctgtctc

SEQ ID NO: 2 - DNA, 66 bp, synthetic construct
  misc_feature 1..66: note = Description of Artificial Sequence: Synthetic oligonucleotide
  modified_base 46..51: mod_base = OTHER; note = a, c, t, g, unknown or other
  modified_base 53..66: mod_base = OTHER; note = a, c, t, g, unknown or other
  source 1..66: mol_type = other DNA
gtggaagaggagaacaatatgctaaatgttgttctcgtctcccacnnnnnncnnnnnnnnnnnnnn

SEQ ID NO: 3 - DNA, 68 bp, synthetic construct
  misc_feature 1..68: note = Description of Artificial Sequence: Synthetic oligonucleotide
  modified_base 50..52: mod_base = OTHER; note = a, c, t, g, unknown or other
  modified_base 54..68: mod_base = OTHER; note = a, c, t, g, unknown or other
  source 1..68: mol_type = other DNA
gggtggaagaggagaacaatatgctaaatgttgttctcgtctcccacctnnncnnnnnnnnnnnnnnn

SEQ ID NO: 4 - DNA, 66 bp, synthetic construct
  misc_feature 1..66: note = Description of Artificial Sequence: Synthetic oligonucleotide
  modified_base 46..51: mod_base = OTHER; note = a, c, t, g, unknown or other
  modified_base 53..66: mod_base = OTHER; note = a, c, t, g, unknown or other
  source 1..66: mol_type = other DNA
ggtgaagaggagaacaatatgctaaatgttgttctcgtctccaccnnnnnncnnnnnnnnnnnnnn

SEQ ID NO: 5 - DNA, 66 bp, synthetic construct
  misc_feature 1..66: note = Description of Artificial Sequence: Synthetic oligonucleotide
  modified_base 46..52: mod_base = OTHER; note = a, c, t, g, unknown or other
  modified_base 54..66: mod_base = OTHER; note = a, c, t, g, unknown or other
  source 1..66: mol_type = other DNA
ggtgaagaggagaacaatatgctaaatgttgttctcgtctccaccnnnnnnncnnnnnnnnnnnnn

SEQ ID NO: 6 - DNA, 66 bp, synthetic construct
  misc_feature 1..66: note = Description of Artificial Sequence: Synthetic oligonucleotide
  modified_base 46..51: mod_base = OTHER; note = a, c, t, g, unknown or other
  modified_base 53..66: mod_base = OTHER; note = a, c, t, g, unknown or other
  source 1..66: mol_type = other DNA
gtggaagaggagaacaataggctaaacgttgttctcgtctcccacnnnnnncnnnnnnnnnnnnnn

SEQ ID NO: 7 - DNA, 68 bp, synthetic construct
  misc_feature 1..68: note = Description of Artificial Sequence: Synthetic oligonucleotide
  modified_base 50..52: mod_base = OTHER; note = a, c, t, g, unknown or other
  modified_base 54..68: mod_base = OTHER; note = a, c, t, g, unknown or other
  source 1..68: mol_type = other DNA
gggtggaagaggagaacaataggctaaacgttgttctcgtctcccacctnnncnnnnnnnnnnnnnnn

SEQ ID NO: 8 - DNA, 66 bp, synthetic construct
  misc_feature 1..66: note = Description of Artificial Sequence: Synthetic oligonucleotide
  modified_base 46..51: mod_base = OTHER; note = a, c, t, g, unknown or other
  modified_base 53..66: mod_base = OTHER; note = a, c, t, g, unknown or other
  source 1..66: mol_type = other DNA
ggtgaagaggagaacaataggctaaacgttgttctcgtctccaccnnnnnncnnnnnnnnnnnnnn

SEQ ID NO: 9 - DNA, 66 bp, synthetic construct
  misc_feature 1..66: note = Description of Artificial Sequence: Synthetic oligonucleotide
  modified_base 46..52: mod_base = OTHER; note = a, c, t, g, unknown or other
  modified_base 54..66: mod_base = OTHER; note = a, c, t, g, unknown or other
  source 1..66: mol_type = other DNA
ggtgaagaggagaacaataggctaaacgttgttctcgtctccaccnnnnnnncnnnnnnnnnnnnn

SEQ ID NO: 10 - DNA, 312 bp, synthetic construct
  misc_feature 1..312: note = Description of Artificial Sequence: Synthetic polynucleotide
  source 1..312: mol_type = other DNA
ggccgggcgcggtggctcacgcctgtaatcccagcactttgggaggccgaggcggggagattgcttgagcccaggagttcgagaccagcctgggcaacatagcgagaccccgtctctacaaaaaatacaaaaattagccgggcgtggtggcgcgcgcctgtagtcccagctactcgggaggctgaggcaggaggatcgcttgagcccaggagttcgaggctgcagtgagctatgatcgcgccactgcactccagcctgggcgacagagcgagaccctgtctcaaaaaaaaaaaaaaaaaaaaaaaaaaaaaa

SEQ ID NO: 11 - DNA, 393 bp, synthetic construct
  misc_feature 1..393: note = Description of Artificial Sequence: Synthetic polynucleotide
  modified_base 117..216: mod_base = OTHER; note = a, c, t, g, unknown or other
  source 1..393: mol_type = other DNA
ggccgggcgcggtggctcacgcctgtaatcccagcactttgggaggccgaggcggggagattgcttgagcccaggagttcgagaccagcctgggcaacatagcgagaccccgtctcnnnnnnnnnnnnnnnnnnnnnnnnnnnnnnnnnnnnnnnnnnnnnnnnnnnnnnnnnnnnnnnnnnnnnnnnnnnnnnnnnnnnnnnnnnnnnnnnnnnnagccgggcgtggtggcgcgcgcctgtagtcccagctactcgggaggctgaggcaggaggatcgcttgagcccaggagttcgaggctgcagtgagctatgatcgcgccactgcactccagcctgggcgacagagcgagaccctgtctcaaaaaaaaaaaaaaaaaaaaaaaaaaaaaa

SEQ ID NO: 12 - RNA, 68 nt, synthetic construct
  misc_feature 1..68: note = Description of Artificial Sequence: Synthetic oligonucleotide
  modified_base 50..52: mod_base = OTHER; note = a, c, u, g, unknown or other
  modified_base 54..68: mod_base = OTHER; note = a, c, u, g, unknown or other
  source 1..68: mol_type = other RNA
gggtggaatagtataacaatatgctaaatgttgttatagtatcccacctnnncnnnnnnnnnnnnnnn

SEQ ID NO: 13 - RNA, 66 nt, synthetic construct
  misc_feature 1..66: note = Description of Artificial Sequence: Synthetic oligonucleotide
  modified_base 46..51: mod_base = OTHER; note = a, c, u, g, unknown or other
  modified_base 53..66: mod_base = OTHER; note = a, c, u, g, unknown or other
  source 1..66: mol_type = other RNA
gtggaatagtataacaatatgctaaatgttgttatagtatcccacnnnnnncnnnnnnnnnnnnnn

SEQ ID NO: 14 - RNA, 76 nt, synthetic construct
  misc_feature 1..76: note = Description of Artificial Sequence: Synthetic oligonucleotide
  modified_base 56..61: mod_base = OTHER; note = a, c, u, g, unknown or other
  modified_base 63..76: mod_base = OTHER; note = a, c, u, g, unknown or other
  source 1..76: mol_type = other RNA
ggtgtcgagaatagtataacaatatgctaaatgttgttatagtatcctcgacaccnnnnnncnnnnnnnnnnnnnn

SEQ ID NO: 15 - RNA, 117 nt, synthetic construct
  misc_feature 1..117: note = Description of Artificial Sequence: Synthetic polynucleotide
  source 1..117: mol_type = other RNA
aactttgtgcattttaggtctcaagtggatattcatggtgtctatgaattcactaaaagatgtcagtgcctggtgaaatcatatacaccatggagaggctataaaatgcagaaggtt

SEQ ID NO: 16 - DNA, 19 bp, synthetic construct
  misc_feature 1..19: note = Description of Artificial Sequence: Synthetic oligonucleotide
  source 1..19: mol_type = other DNA
aaccgagcggtgtctgtga

SEQ ID NO: 17 - DNA, 19 bp, synthetic construct
  misc_feature 1..19: note = Description of Artificial Sequence: Synthetic oligonucleotide
  source 1..19: mol_type = other DNA
aaccgagcggtgtctgtga

SEQ ID NO: 18 - DNA, 19 bp, synthetic construct
  misc_feature 1..19: note = Description of Artificial Sequence: Synthetic oligonucleotide
  source 1..19: mol_type = other DNA
aaccgagcggtgtctgtga

SEQ ID NO: 19 - DNA, 21 bp, synthetic construct
  misc_feature 1..21: note = Description of Artificial Sequence: Synthetic oligonucleotide
  source 1..21: mol_type = other DNA
acaaaccgagcggtgtctgtg

SEQ ID NO: 20 - DNA, 21 bp, synthetic construct
  misc_feature 1..21: note = Description of Artificial Sequence: Synthetic oligonucleotide
  source 1..21: mol_type = other DNA
acaaaccgagcggtgtctgtg

SEQ ID NO: 21 - DNA, 21 bp, synthetic construct
  misc_feature 1..21: note = Description of Artificial Sequence: Synthetic oligonucleotide
  source 1..21: mol_type = other DNA
acaaaccgagcggtgtctgtg

SEQ ID NO: 22 - DNA, 21 bp, synthetic construct
  misc_feature 1..21: note = Description of Artificial Sequence: Synthetic oligonucleotide
  source 1..21: mol_type = other DNA
acaaaccgagcggtgtctgtg

SEQ ID NO: 23 - DNA, 21 bp, synthetic construct
  misc_feature 1..21: note = Description of Artificial Sequence: Synthetic oligonucleotide
  source 1..21: mol_type = other DNA
tacaaaccgagcggtgtctgt

SEQ ID NO: 24 - DNA, 21 bp, synthetic construct
  misc_feature 1..21: note = Description of Artificial Sequence: Synthetic oligonucleotide
  source 1..21: mol_type = other DNA
acaaaccgagcggtgtctgtg

SEQ ID NO: 25 - DNA, 21 bp, synthetic construct
  misc_feature 1..21: note = Description of Artificial Sequence: Synthetic oligonucleotide
  source 1..21: mol_type = other DNA
tacaaaccgagcggtgtctgt

SEQ ID NO: 26 - DNA, 18 bp, synthetic construct
  misc_feature 1..18: note = Description of Artificial Sequence: Synthetic oligonucleotide
  source 1..18: mol_type = other DNA
tacaaaccgagcggtgtc

SEQ ID NO: 27 - DNA, 18 bp, synthetic construct
  misc_feature 1..18: note = Description of Artificial Sequence: Synthetic oligonucleotide
  source 1..18: mol_type = other DNA
tacaaaccgagcggtgtc

SEQ ID NO: 28 - DNA, 18 bp, synthetic construct
  misc_feature 1..18: note = Description of Artificial Sequence: Synthetic oligonucleotide
  source 1..18: mol_type = other DNA
tacaaaccgagcggtgtc

SEQ ID NO: 29 - DNA, 20 bp, synthetic construct
  misc_feature 1..20: note = Description of Artificial Sequence: Synthetic oligonucleotide
  source 1..20: mol_type = other DNA
caaaccgagcggtgtctgtg

SEQ ID NO: 30 - DNA, 20 bp, synthetic construct
  misc_feature 1..20: note = Description of Artificial Sequence: Synthetic oligonucleotide
  source 1..20: mol_type = other DNA
tacaaaccgagcggtgtctg

SEQ ID NO: 31 - DNA, 20 bp, synthetic construct
  misc_feature 1..20: note = Description of Artificial Sequence: Synthetic oligonucleotide
  source 1..20: mol_type = other DNA
tttacaaaccgagcggtgtc

SEQ ID NO: 32 - DNA, 21 bp, synthetic construct
  misc_feature 1..21: note = Description of Artificial Sequence: Synthetic oligonucleotide
  source 1..21: mol_type = other DNA
acaaaccgagcggtgtctgtg

SEQ ID NO: 33 - DNA, 21 bp, synthetic construct
  misc_feature 1..21: note = Description of Artificial Sequence: Synthetic oligonucleotide
  source 1..21: mol_type = other DNA
acaaaccgagcggtgtctgtg

SEQ ID NO: 34 - DNA, 21 bp, synthetic construct
  misc_feature 1..21: note = Description of Artificial Sequence: Synthetic oligonucleotide
  source 1..21: mol_type = other DNA
acaaaccgagcggtgtctgtg

SEQ ID NO: 35 - RNA, 120 nt, synthetic construct
  misc_feature 1..120: note = Description of Artificial Sequence: Synthetic polynucleotide
  modified_base 46..59: mod_base = OTHER; note = a, c, u, g, unknown or other
  modified_base 61..75: mod_base = OTHER; note = a, c, u, g, unknown or other
  source 1..120: mol_type = other RNA
gtggaatagtataacaatatgctaaatgttgttatagtatcccacnnnnnnnnnnnnnncnnnnnnnnnnnnnnncaccctatgatattgttgtaaatcgtataacaatatgataaggtg

SEQ ID NO: 36 - skipped

SEQ ID NO: 37 - RNA, 66 nt, synthetic construct; identical to SEQ ID NO: 13
  misc_feature 1..66: note = Description of Artificial Sequence: Synthetic oligonucleotide
  modified_base 46..51: mod_base = OTHER; note = a, c, u, g, unknown or other
  modified_base 53..66: mod_base = OTHER; note = a, c, u, g, unknown or other
  source 1..66: mol_type = other RNA

SEQ ID NO: 38 - DNA, 283 bp, synthetic construct
  misc_feature 1..283: note = Description of Artificial Sequence: Synthetic polynucleotide
  source 1..283: mol_type = other DNA
ggccgggcgcggtggctcacgcctgtaatcccagcactttgggaggccgaggcggggagattgcttgagcccaggagttcgagaccagcctgggcaacatagcgagaccccgtctcatactgccgccagctggattagccgggcgtggtggcgcgcgcctgtagtcccagctactcgggaggctgaggcaggaggatcgcttgagcccaggagttcgaggctgcagtgagctatgatcgcgccactgcactccagcctgggcgacagagcgagaccctgtctc

SEQ ID NO: 39 - DNA, 303 bp, synthetic construct
  misc_feature 1..303: note = Description of Artificial Sequence: Synthetic polynucleotide
  source 1..303: mol_type = other DNA
ggccgggcgcggtggctcacgcctgtaatcccagcactttgggaggccgaggcggggagattgcttgagcccaggagttcgagaccagcctgggcaacatagcgagaccccgtctcactgtacagaatactgccgccagctggatttcccaattctagccgggcgtggtggcgcgcgcctgtagtcccagctactcgggaggctgaggcaggaggatcgcttgagcccaggagttcgaggctgcagtgagctatgatcgcgccactgcactccagcctgggcgacagagcgagaccctgtctc

SEQ ID NO: 40 - DNA, 322 bp, synthetic construct
  misc_feature 1..322: note = Description of Artificial Sequence: Synthetic polynucleotide
  source 1..322: mol_type = other DNA
ggccgggcgcggtggctcacgcctgtaatcccagcactttgggaggccgaggcggggagattgcttgagcccaggagttcgagaccagcctgggcaacatagcgagaccccgtctctcttgtgtctactgtacagaatactgccgccagctggatttcccaattctgagtaacacagccgggcgtggtggcgcgcgcctgtagtcccagctactcgggaggctgaggcaggaggatcgcttgagcccaggagttcgaggctgcagtgagctatgatcgcgccactgcactccagcctgggcgacagagcgagaccctgtctc

SEQ ID NO: 41 - DNA, 363 bp, synthetic construct
  misc_feature 1..363: note = Description of Artificial Sequence: Synthetic polynucleotide
  source 1..363: mol_type = other DNA
ggccgggcgcggtggctcacgcctgtaatcccagcactttgggaggccgaggcggggagattgcttgagcccaggagttcgagaccagcctgggcaacatagcgagaccccgtctctgataaaaggcgtacataattcttgtgtctactgtacagaatactgccgccagctggatttcccaattctgagtaacactctgcaatccaaacagggttcagccgggcgtggtggcgcgcgcctgtagtcccagctactcgggaggctgaggcaggaggatcgcttgagcccaggagttcgaggctgcagtgagctatgatcgcgccactgcactccagcctgggcgacagagcgagaccctgtctc

SEQ ID NO: 42 - protein, 386 aa, synthetic construct
  REGION 1..386: note = Description of Artificial Sequence: Synthetic polypeptide
QLHLPQVLADAVSRLVLGKFGDLTDNFSSPHARRKVLAGVVMTTGTDVKDAKVISVSTGTKCINGEYMSDRGLALNDCHAEIISRRSLLRFLYTQLELYLNNKDDQKRSIFQKSERGGFRLKENVQFHLYISTSPCGDARIFSPHEPIIEEPADRHPNRKARGQLRTKIESGEGTIPVRSNASIQTWDGVLQGERLLTMSCSDKIARWNVVGIQGSLLSIFVEPIYFSSIILGSLYHGDHLSRAMYQRISNIEDLPPLYTLNKPLLSGISNAEARQPGKAPNFSVNWTVGDSAIEVINATTGKDELGRASRLCKHALYCRWMRVHGKVPSHLLRSKITKPNVYHESKLAAKEYQAAKARLFTAFIKAGLGAWVEKPTEQDQFSLTP

SEQ ID NO: 43 - DNA, 1662 bp, synthetic construct
  misc_feature 1..1662: note = Description of Artificial Sequence: Synthetic polynucleotide
  source 1..1662: mol_type = other DNA
atgaagaccttaattcttgccgttgcattagtctactgcgccactgttcattgccaggactgtccttacgaacctgatccaccaaacacagttccaacttcctgtgaagctaaagaaggagaatgtattgatagcagctgtggcacctgcacgagagacatactatcagatggactgtgtgaaaataaaccaggaaaaacatgttgccgaatgtgtcagtatgtaattgaatgcagagtagaggccgcaggatagtttagaacattctatggaaagagattccagttccaggaacctggtacatacgtgttgggtcaaggaaccaagggcggcgactggaaggtgtccatcaccctggagaacctggatggaaccaagggggctgtgctgaccaagacaagactggaagtggctggagacatcattgacatcgctcaagctactgagaatcccatcactgtaaacggtggagctgaccctatcatcgccaacccgtacaccatcggcgaggtcaccatcgctgttgttgagatgccaggcttcaacatcaccgtcattgagttcttcaaactgatcgtgatcgacatcctcggaggaagatctgtaagaatcgccccagacacagcaaacaaaggaatgatctctggcctctgtggagatcttaaaatgatggaagatacagacttcacttcagatccagaacaactcgctattcagcctaagatcaaccaggagtttgacggttgtccactctatggaaatcctgatgacgttgcatactgcaaaggtcttctggagccgtacaaggacagctgccgcaaccccatcaacttctactactacaccatctcctgcgccttcgcccgctgtatgggtggagacgagcgagcctcacacgtgctgcttgactacagggagacgtgcgctgctcccgaaactagaggaacctgcgttttgtctggacatactttctacgatacatttgacaaagcaagataccaattccagggtccctgcaaggagattcttatggccgccgactgtttctggaacacttgggatgtgaaggtttcacacaggaatgttgactcttacactgaagtagagaaagtacgaatcaggaaacaatcgactgtagtagaactcattgttgatggaaaacagattctggttggaggagaagccgtgtccgtcccgtacagctctcagaacacttccatctactggcaagatggtgacatactgactacagccatcctacctgaagctctggtggtcaagttcaacttcaagcaactgctcgtcgtacatattagagatccattcgatggtaagacttgcggtatttgcggtaactacaaccaggatttcagtgatgattcttttgatgctgaaggagcctgtgatctgacccccaacccaccgggatgcaccgaagaacagaaacctgaagctgaacgactctgcaatagtctcttcgccggtcaaagtgatcttgatcagaaatgtaacgtgtgccacaagcctgaccgtgtcgaacgatgcatgtacgagtattgcctgaggggacaacagggtttctgtgaccacgcatgggagttcaagaaagaatgctacataaagcatggagacaccctagaagtaccagatgaatgcaaataa

SEQ ID NO: 44 - DNA, 61 bp, synthetic construct
  misc_feature 1..61: note = Description of Artificial Sequence: Synthetic oligonucleotide
  source 1..61: mol_type = other DNA
ggccctgaaaaagggcctgttctaaaccatcctgcggcctcaacatgaggatcacccatgc

SEQ ID NO: 45 - DNA, 64 bp, synthetic construct
  misc_feature 1..64: note = Description of Artificial Sequence: Synthetic oligonucleotide
  source 1..64: mol_type = other DNA
aacatgaggatcacccatgtcctaaaccatcctgcggcctctactctggccctgaaaaagggcc

SEQ ID NO: 46 - DNA, 62 bp, synthetic construct
  misc_feature 1..62: note = Description of Artificial Sequence: Synthetic oligonucleotide
  source 1..62: mol_type = other DNA
aacatgaggatcacccatgtcctaaaccatcctgcggcctcaacatgaggatcacccatgtc

SEQ ID NO: 47 - DNA, 64 bp, synthetic construct
  misc_feature 1..64: note = Description of Artificial Sequence: Synthetic oligonucleotide
  source 1..64: mol_type = other DNA
ggccctgaaaaagggcctgttctaaaccatcctgcggcctctactctggccctgaaaaagggcc

SEQ ID NO: 48 - protein, 317 aa, synthetic construct
  REGION 1..317: note = Description of Artificial Sequence: Synthetic polypeptide
MLPPLERLTLGSDYKDDDDKGSGSGSMASNFTQFVLVDNGGTGDVTVAPSNFANGIAEWISSNSRSQAYKVTCSVRQSSAQNRKYTIKVEVPKGAWRSYLNMELTIPIFATNSDCELIVKAMQGLLKDGNPIPSAIAANSGIYGGSGSGAGSGSPAGGGAPGSGGGSQLHLPQVLADAVSRLVLGKFGDLTDNFSSPHARRKVLAGVVMTTGTDVKDAKVISVSTGTKCINGEYMSDRGLALNDCHAEIISRRSLLRFLYTQLELYLNNKDDQKRSIFQKSERGGFRLKENVQFHLYISTSPCGDARIFSPHEPILE

SEQ ID NO: 49 - protein, 412 aa, synthetic construct
  REGION 1..412: note = Description of Artificial Sequence: Synthetic polypeptide
MEPADRHPNRKARGQLRTKIESGEGTIPVRSNASIQTWDGVLQGERLLTMSCSDKIARWNVVGIQGSLLSIFVEPIYFSSIILGSLYHGDHLSRAMYQRISNIEDLPPLYTLNKPLLSGISNAEARQPGKAPNFSVNWTVGDSAIEVINATTGKDELGRASRLCKHALYCRWMRVHGKVPSHLLRSKITKPNVYHESKLAAKEYQAAKARLFTAFIKAGLGAWVEKPTEQDQFSLTPGGSGSGAGSGSPAGGGAPGSGGGSNARTRRRERRAEKQAQWKAANGGGGSGGGGSGGGGSNARTRRRERRAEKQAQWKAANGGGGSGGGGSGGGGSNARTRRRERRAEKQAQWKAANGGGGSGGGGSGGGGSNARTRRRERRAEKQAQWKAANGSYPYDVPDYAGSLPPLERLTL

SEQ ID NO: 50 - protein, 320 aa, synthetic construct
  REGION 1..320: note = Description of Artificial Sequence: Synthetic polypeptide
MLPPLERLTLGSDYKDDDDKGSGSGSMASNFTQFVLVDNGGTGDVTVAPSNFANGIAEWISSNSRSQAYKVTCSVRQSSAQNRKYTIKVEVPKGAWRSYLNMELTIPIFATNSDCELIVKAMQGLLKDGNPIPSAIAANSGIYGGSGSGAGSGSPAGGGAPGSGGGSQLHLPQVLADAVSRLVLGKFGDLTDNFSSPHARRKVLAGVVMTTGTDVKDAKVISVSTGTKCINGEYMSDRGLALNDCHAEIISRRSLLRFLYTQLELYLNNKDDQKRSIFQKSERGGFRLKENVQFHLYISTSPCGDARIFSPHEPILEEPA

SEQ ID NO: 51 - protein, 409 aa, synthetic construct
  REGION 1..409: note = Description of Artificial Sequence: Synthetic polypeptide
MDRHPNRKARGQLRTKIESGEGTIPVRSNASIQTWDGVLQGERLLTMSCSDKIARWNVVGIQGSLLSIFVEPIYFSSIILGSLYHGDHLSRAMYQRISNIEDLPPLYTLNKPLLSGISNAEARQPGKAPNFSVNWTVGDSAIEVINATTGKDELGRASRLCKHALYCRWMRVHGKVPSHLLRSKITKPNVYHESKLAAKEYQAAKARLFTAFIKAGLGAWVEKPTEQDQFSLTPGGSGSGAGSGSPAGGGAPGSGGGSNARTRRRERRAEKQAQWKAANGGGGSGGGGSGGGGSNARTRRRERRAEKQAQWKAANGGGGSGGGGSGGGGSNARTRRRERRAEKQAQWKAANGGGGSGGGGSGGGGSNARTRRRERRAEKQAQWKAANGSYPYDVPDYAGSLPPLERLTL

SEQ ID NO: 52 - protein, 317 aa, synthetic construct
  REGION 1..317: note = Description of Artificial Sequence: Synthetic polypeptide
MLPPLERLTLGSDYKDDDDKGSGSGSMASNFTQFVLVDNGGTGDVTVAPSNFANGIAEWISSNSRSQAYKVTCSVRQSSAQNRKYTIKVEVPKGAWRSYLNMELTIPIFATNSDCELIVKAMQGLLKDGNPIPSAIAANSGIYGGSGSGAGSGSPAGGGAPGSGGGSQLHLPQVLADAVSRLVIGKFGDLTDNFSSPHARRIGLAGVVMTTGTDVKDAKVICVSTGSKCINGEYLSDRGLALNDCHAEIVSRRSLLRFLYTQLELYLNNEDDQKRSIFQKSERGGFRLKENIQFHLYISTSPCGDARIFSPHEAILE

SEQ ID NO: 53 - protein, 412 aa, synthetic construct
  REGION 1..412: note = Description of Artificial Sequence: Synthetic polypeptide
MEPADRHPNRKARGQLRTKIEAGQGTIPVRNNASIQTWDGVLQGERLLTMSCSDKIARWNVVGIQGSLLSIFVEPIYFSSIILGSLYHGDHLSRAMYQRISNIEDLPPLYTLNKPLLTGISNAEARQPGKAPIFSVNWTVGDSAIEVINATTGKGELGRASRLCKHALYCRWMRVHGKVPSHLLRSKITKPNVYHETKLAAKEYQAAKARLFTAFIKAGLGAWVEKPTEQDQFSLTPGGSGSGAGSGSPAGGGAPGSGGGSNARTRRRERRAEKQAQWKAANGGGGSGGGGSGGGGSNARTRRRERRAEKQAQWKAANGGGGSGGGGSGGGGSNARTRRRERRAEKQAQWKAANGGGGSGGGGSGGGGSNARTRRRERRAEKQAQWKAANGSYPYDVPDYAGSLPPLERLTL

SEQ ID NO: 54 - protein, 320 aa, synthetic construct
  REGION 1..320: note = Description of Artificial Sequence: Synthetic polypeptide
MLPPLERLTLGSDYKDDDDKGSGSGSMASNFTQFVLVDNGGTGDVTVAPSNFANGIAEWISSNSRSQAYKVTCSVRQSSAQNRKYTIKVEVPKGAWRSYLNMELTIPIFATNSDCELIVKAMQGLLKDGNPIPSAIAANSGIYGGSGSGAGSGSPAGGGAPGSGGGSQLHLPQVLADAVSRLVIGKFGDLTDNFSSPHARRIGLAGVVMTTGTDVKDAKVICVSTGSKCINGEYLSDRGLALNDCHAEIVSRRSLLRFLYTQLELYLNNEDDQKRSIFQKSERGGFRLKENIQFHLYISTSPCGDARIFSPHEAILEEPA

SEQ ID NO: 55 - protein, 409 aa, synthetic construct
  REGION 1..409: note = Description of Artificial Sequence: Synthetic polypeptide
MDRHPNRKARGQLRTKIEAGQGTIPVRNNASIQTWDGVLQGERLLTMSCSDKIARWNVVGIQGSLLSIFVEPIYFSSIILGSLYHGDHLSRAMYQRISNIEDLPPLYTLNKPLLTGISNAEARQPGKAPIFSVNWTVGDSAIEVINATTGKGELGRASRLCKHALYCRWMRVHGKVPSHLLRSKITKPNVYHETKLAAKEYQAAKARLFTAFIKAGLGAWVEKPTEQDQFSLTPGGSGSGAGSGSPAGGGAPGSGGGSNARTRRRERRAEKQAQWKAANGGGGSGGGGSGGGGSNARTRRRERRAEKQAQWKAANGGGGSGGGGSGGGGSNARTRRRERRAEKQAQWKAANGGGGSGGGGSGGGGSNARTRRRERRAEKQAQWKAANGSYPYDVPDYAGSLPPLERLTL

SEQ ID NO: 56 - RNA, 11 nt, synthetic construct
  misc_feature 1..11: note = Description of Artificial Sequence: Synthetic oligonucleotide
  source 1..11: mol_type = other RNA
attgcactccg

SEQ ID NO: 57 - protein, 393 aa, synthetic construct
  REGION 1..393: note = Description of Artificial Sequence: Synthetic polypeptide
MASNFTQFVLVDNGGTGDVTVAPSNFANGIAEWISSNSRSQAYKVTCSVRQSSAQNRKYTIKVEVPKGAWRSYLNMELTIPIFATNSDCELIVKAMQGLLKDGNPIPSAIAANSGIYGGSGSGAGSGSPAGGGAPGSGGGSSGSETPGTSESATPESMTSEKGPSTGDPTLRRRIEPWEFDVFYDPRELRKEACLLYEIKWGMSRKIWRSSGKNTTNHVEVNFIKKFTSERDFHPSMSCSITWFLSWSPCWECSQAIREFLSRHPGVTLVIYVARLFWHMDQQNRQGLRDLVNSGVTIQIMRASEYYHCWRNFVNYPPGDEAHWPQYPPLWMMLYALELHCIILSLPPCLKISRRWQNHLTFFRLHLQNCHYQTIPPHILLATGLIHPSVAWR

SEQ ID NO: 58 - protein, 365 aa, synthetic construct
  REGION 1..365: note = Description of Artificial Sequence: Synthetic polypeptide
MASNFTQFVLVDNGGTGDVTVAPSNFANGIAEWISSNSRSQAYKVTCSVRQSSAQNRKYTIKVEVPKGAWRSYLNMELTIPIFATNSDCELIVKAMQGLLKDGNPIPSAIAANSGIYGGSGSGAGSGSPAGGGAPGSGGGSMAQKEEAAVATEAASQNGEDLENLDDPEKLKELIELPPFEIVTGERLPANFFKFQFRNVEYSSGRNKTFLCYVVEAQGKGGQVQASRGYLEDEHAAAHAEEAFFNTILPAFDPALRYNVTWYVSSSPCAACADRIIKTLSKTKNLRLLILVGRLFMWEEPEIQAALKKLKEAGCKLRIMKPQDFEYVWQNFVEQEEGESKAFQPWEDIQENFLYYEEKLADILK

SEQ ID NO: 59 - protein, 340 aa, synthetic construct
  REGION 1..340: note = Description of Artificial Sequence: Synthetic polypeptide
MASNFTQFVLVDNGGTGDVTVAPSNFANGIAWWISSNSRSQAYKVTCSVRQSSAQNRKYTIKVEVPKGAWRSYLNMELTIPIFATNSDCELIVKAMQGLLKDGNPIPSAIAANSGIYGGSGSGAGSGSPAGGGAPGSGGGSMEASPASGPRHLMDPHIFTSNFNNGIGRHKTYLCYEVERLDNGTSVKMDQHRGFLHNQAKNLLCGFYGRHAELRFLDLVPSLQLDPAQIYRVTWFISWSPCFSWGCAGEVRAFLQENTHVRLRIFAARIYDYDPLYKEALQMLRDAGAQVSIMTYDEFKHCWDTFVDHQGCPFQPWDGLDEHSQALSGRLRAILQNQGN

SEQ ID NO: 60 - protein, 523 aa, synthetic construct
  REGION 1..523: note = Description of Artificial Sequence: Synthetic polypeptide
MASNFTQFVLVDNGGTGDVTVAPSNFANGIAEWISSNSRSQAYKVTCSVRQSSAQNRKYTIKVEVPKGAWRSYLNMELTIPIFATNSDCELIVKAMQGLLKDGNPIPSAIAANSGIYGGSGSGAGSGSPAGGGAPGSGGGSMNPQIRNPMERMYRDTFYDNFENEPILYGRSYTWLCYEVKIKRGRSNLLWDTGVFRGQVYFKPQYHAEMCFLSWFCGNQLPAYKCFQITWFVSWTPCPDCVAKLAEFLSEHPNVTLTISAARLYYYWERDYRRALCRLSQAGARVTIMDYEEFAYCWENFVYNEGQQFMPWYKFDENYAFLHRTLKEILRYLMDPDTFTFNFNNDPLVLRRRQTYLCYEVERLDNGTWVLMDQHMGFLCNEAKNLLCGFYGRHAELRFLDLVPSLQLDPAQIYRVTWFISWSPCFSWGCAGEVRAFLQENTHVRLRIFAARIYDYDPLYKEALQMLRDAGAQVSIMTYDEFEYCWFTFVYRQGCPFQPWDGLEEHSQALSGRLRAILQNQGN

SEQ ID NO: 61 - protein, 331 aa, synthetic construct
  REGION 1..331: note = Description of Artificial Sequence: Synthetic polypeptide
MASNFTQFVLVDNGGTGDVTVAPSNFANGIAEWISSNSRSQAYKVTCSVRQSSAQNRKYTIKVEVPKGAWRSYLNMELTIPIFATNSDCELIVKAMQGLLKDGNPIPSAIAANSGIYGGSGSGAGSGSPAGGGAPGSGGGSMNPQIRNPMKAMYPGTFYFQFKNLWEANDRNETWLCFTVEGIKRRSVVSWKTGVFRNQVDSETHCHAERCFLSWFCDDILSPNTKYQVTWYTSWSPCPDCAGEVAEFLARHSNVNLTIFTARLYYFQYPCYQEGLRSLSQEGVAVEIMDYEDFKYCWENFVYNDNEPFKPWKGLKTNFRLLKRRLRESLQ

SEQ ID NO: 62 - protein, 527 aa, synthetic construct
  REGION 1..527: note = Description of Artificial Sequence: Synthetic polypeptide
MASNFTQFVLVDNGGTGDVTVAPSNFANGIAEWISSNSRSQAYKVTCSVRQSSAQNRKYTIKVEVPKGAWRSYLNMELTIPIFATNSDCELIVKAMQGLLKDGNPIPSAIAANSGIYGGSGSGAGSGSPAGGGAPGSGGGSMNPQIRNPMERMYRDTFYDNFENEPILYGRSYTWLCYEVKIKRGRSNLLWDTGVFRGPVLPKRQSNHRQEVYFRFENHAEMCFLSWFCGNRLPANRRFQITWFVSWNPCLPCVVKVTKFLAEHPNVTLTISAARLYYYRDRDWRWVLLRLHKAGARVKIMDYEDFAYCWENFVCNEGQPFMPWYKFDDNYASLHRTLKEILRNPMEAMYPHIFYFHFKNLLKACGRNESWLCFTMEVTKHHSAVFRKRGVFRNQVDPETHCHAERCFLSWFCDDILSPNTNYEVTWYTSWSPCPECAGEVAEFLARHSNVNLTIFTARLCYFWDTDYQEGLCSLSQEGASVKIMGYKDFVSCWKNFVYSDDEPFKPWKGLQTNFRLLKRRLREILQ

SEQ ID NO: 63 - protein, 514 aa, synthetic construct
  REGION 1..514: note = Description of Artificial Sequence: Synthetic polypeptide
MASNFTQFVLVDNGGTGDVTVAPSNFANGIAEWISSNSRSQAYKVTCSVRQSSAQNRKYTIKVEVPKGAWRSYLNMELTIPIFATNSDCELIVKAMQGLLKDGNPIPSAIAANSGIYGGSGSGAGSGSPAGGGAPGSGGGSMKPHFRNTVERMYRDTFSYNFYNRPILSRRNTVWLCYEVKTKGPSRPRLDAKIFRGQVYSQPEHHAEMCFLSWFCGNQLPAYKCFQITWFVSWTPCPDCVAKLAEFLAEHPNVTLTISAARLYYYWERDYRRALCRLSQAGARVKIMDDEEFAYCWENFVYSEGQPFMPWYKFDDNYAFLHRTLKEILRNPMEAMYPHIFYFHFKNLRKAYGRNESWLCFTMEVVKHHSPVSWKRGVFRNQVDPETHCHAERCFLSWFCDDILSPNTNYEVTWYTSWSPCPECAGEVAEFLARHSNVNLTIFTARLYYFWDTDYQEGLRSLSQEGASVEIMGYKDFKYCWENFVYNDDEPFKPWKGLKYNFLFLDSKLQEILE

SEQ ID NO: 64 - protein, 525 aa, synthetic construct
  REGION 1..525: note = Description of Artificial Sequence: Synthetic polypeptide
MASNFTQFVLVDNGGTGDVTVAPSNFANGIAEWISSNSRSQAYKVTCSVRQSSAQNRKYTIKVEVPKGAWRSYLNMELTIPIFATNSDCELIVKAMQGLLKDGNPIPSAIAANSGIYGGSGSGAGSGSPAGGGAPGSGGGSMKPHFRNTVERMYRDTFSYNFYNRPILSRRNTVWLCYEVKTKGPSRPPLDAKIFRGQVYSELKYHPEMRFFHWFSKWRKLHRDQEYEVTWYISWSPCTKCTRDMATFLAEDPKVTLTIFVARLYYFWDPDYQEALRSLCQKRDGPRATMKIMNYDEFQHCWSKFVYSQRELFEPWNNLPKYYILLHIMLGEILRHSMDPPTFTFNFNNEPWVRGRHETYLCYEVERMHNDTWVLLNQRRGFLCNQAPHKHGFLEGRHAELCFLDVIPFWKLDLDQDYRVTCFTSWSPCFSCAQEMAKFISKNKHVSLCIFTARIYDDQGRCQEGLRTLAEAGAKISIMTYSEFKHCWDTFVDHQGCPFQPWDGLDEHSQDLSGRLRAILQNQEN

SEQ ID NO: 65 - protein, 341 aa, synthetic construct
  REGION 1..341: note = Description of Artificial Sequence: Synthetic polypeptide
MASNFTQFVLVDNGGTGDVTVAPSNFANGIAEWISSNSRSQAYKVTCSVRQSSAQNRKYTIKVEVPKGAWRSYLNMELTIPIFATNSDCELIVKAMQGLLKDGNPIPSAIAANSGIYGGSGSGAGSGSPAGGGAPGSGGGSMALLTAETFRLQFNNKRRLRRPYYPRKALLCYQLTPQNGSTPTRGYFENKKKCHAEICFINEIKSMGLDETQCYQVTCYLTWSPCSSCAWELVDFIKAHDHLNLGIFASRLYYHWCKPQQKGLRLLCGSQVPVEVMGFPEFADCWENFVDHEKPLSFNPYKMLEELDKNSRAIKRRLERIKIPGVRAQGRYMDILCDAEV

SEQ ID NO: 66 - protein, 508 aa, synthetic construct
  REGION 1..508: note = Description of Artificial Sequence: Synthetic polypeptide
MASNFTQFVLVDNGGTGDVTVAPSNFANGIAEWISSNSRSQAYKVTCSVRQSSAQNRKYTIKVEVPKGAWRSYLNMELTIPIFATNSDCELIVKAMQGLLKDGNPIPSAIAANSGIYGGSGSGAGSGSPAGGGAPGSGGGSMEPIYEEYLANHGTIVKPYYWLSFSLDCSNCPYHIRTGEEARVSLTEFCQIFGFPYGTTFPQTKHLTFYELKTSSGSLVQKGHASSCTGNYIHPESMLFEMNGYLDSAIYNNDSIRHIILYSNNSPCNEANHCCISKMYNFLITYPGITLSIYFSQLYHTEMDFPASAWNREALRSLASLWPRVVLSPISGGIWHSVLHSFISGVSGSHVFQPILTGRALADRHNAYEINAITGVKPYFTDVLLQTKRNPNTKAQEALESYPLNNAFPGQFFQMPSGQLQPNLPPDLRAPVVFVLVPLRDLPPMHMGQNPNKPRNIVRHLNMPQMSFQETKDLGRLPTGRSVEIVEITEQFASSKEADEKKKKKGKK

SEQ ID NO: 67 - protein, 339 aa, synthetic construct
  REGION 1..339: note = Description of Artificial Sequence: Synthetic polypeptide
MASNFTQFVLVDNGGTGDVTVAPSNFANGIAEWISSNSRSQAYKVTCSVRQSSAQNRKYTIKVEVPKGAWRSYLNMELTIPIFATNSDCELIVKAMQGLLKDGNPIPSAIAANSGIYGGSGSGAGSGSPAGGGAPGSGGGSMDSLLMNRRKFLYQFKNVRWAKGRRETYLCYVVKRRDSATSFSLDFGYLRNKNGCHVELLFLRYISDWDLDPGRCYRVTWFTSWSPCYDCARHVADFLRGNPNLSLRIFTARLYFCEDRKAEPEGLRRLHRAGVQIAIMTFKDYFYCWNTFVENHERTFKAWEGLHENSVRLSRQLRRILLPLYEVDDLRDAFRTLGL

SEQ ID NO: 68 - protein, 643 aa, synthetic construct
  REGION 1..643: note = Description of Artificial Sequence: Synthetic polypeptide
MASNFTQFVLVDNGGTGDVTVAPSNFANGIAEWISSNSRSQAYKVTCSVRQSSAQNRKYTIKVEVPKGAWRSYLNMELTIPIFATNSDCELIVKAMQGLLKDGNPIPSAIAANSGIYGGSGSGAGSGSPAGGGAPGSGGGSMWTADEIAQLCYEHYGIRLPKKGKPEPNHEWTLLAAVVKIQSPADKACDTPDKPVQVTKEVVSMGTGTKCIGQSKMRKNGDILNDSHAEVIARRSFQRYLLHQLQLAATLKEDSIFVPGTQKGVWKLRRDLIFVFFSSHTPCGDASIIPMLEFEDQPCCPVFRNWAHNSSVEASSNLEAPGNERKCEDPDSPVTKKMRLEPGTAAREVTNGAAHHQSFGKQKSGPISPGIHSCDLTVEGLATVTRIAPGSAKVIDVYRTGAKCVPGEAGDSGKPGAAFHQVGLLRVKPGRGDRTRSMSCSDKMARWNVLGCQGALLMHLLEEPIYLSAVVIGKCPYSQEAMQRALIGRCQNVSALPKGFGVQELKILQSDLLFEQSRSAVQAKRADSPGRLVPCGAAISWSAVPEQPLDVTANGFPQGTTKKTIGSLQARSQISKVELFRSFQKLLSRIARDKWPHSLRVQKLDTYQEYKEAASSYQEAWSTLRKQVFGSWIRNPPDYHQFK

SEQ ID NO: 69 - DNA, 741 bp, synthetic construct
  misc_feature 1..741: note = Description of Artificial Sequence: Synthetic polynucleotide
  source 1..741: mol_type = other DNA
atggtgagcaagggcgaggagctgttcaccggggtggtgcccatcctggtcgagctggacggcgacgtaaacggccacaagttcagcgtgtccggcgagggcgagggcgatgccacctacggcaagctgaccctgaagttcatctgcaccaccggcaagctgcccgtgccctggcccaccctcgtgaccaccctgacctacggcgtgcagtgcttcagccgctaccccgaccacatgaagcagcacgacttcttcaagtccgccatgcccgaaggctacgtccaggagcgcaccatcttcttcaaggacgacggcaactacaagacccgcgccgaggtgaagttcgagggcgacaccctggtgaaccgcatcgagctgaagggcatcgacttcaaggaggacggcaacatcctggggcacaagctggagtacaactacaacagccacaacgtctatatcatggccgacaagcagaagaacggcatcaaggtgaacttcaagatccgccacaacatcgaggacggcagcgtgcagctcgccgaccactaccagcagaacacccccatcggcgacggccccgtgctgctgcccgacaatcattattcgagcactcagtccgccctgagcaaagaccccaacgagaagcgcgatcacatggtcctgctggagttcgtgaccgccgccgggatcactctcggcatggacgagctgtacaagtactcagatctcgagctcaagtag

SEQ ID NO: 70 - DNA, 140 bp, synthetic construct
  misc_feature 1..140: note = Description of Artificial Sequence: Synthetic polynucleotide
  source 1..140: mol_type = other DNA
gcgcctccatcgaagtgtaaagccatctatcgatgggaaagtctttgctctccccggacactctgctccttaaatgaaacacgggctcgtgcacggggccaaagcgcctccatcgaagtgtaaagccatctatcgatggg

SEQ ID NO: 71 - DNA, 98 bp, synthetic construct
  misc_feature 1..98: note = Description of Artificial Sequence: Synthetic oligonucleotide
  source 1..98: mol_type = other DNA
gccatctatcgatgggaaagtctttgctctccccggacactctgctccttaaatgaaacacgggctcgtgcacggggccaaagccatctatcgatggg

SEQ ID NO: 72 - DNA, 68 bp, synthetic construct
  misc_feature 1..68: note = Description of Artificial Sequence: Synthetic oligonucleotide
  source 1..68: mol_type = other DNA
gccatctatcgatgggaaacggactgagtgctcaaaatgattgtcgggcaaagccatctatcgatggg

SEQ ID NO: 73 - DNA, 78 bp, synthetic construct
  misc_feature 1..78: note = Description of Artificial Sequence: Synthetic oligonucleotide
  source 1..78: mol_type = other DNA
gccatctatcgatgggaaatgctcagggcggactgagaaaattgtcgggcagcagcacgaaagccatctatcgatggg

SEQ ID NO: 74 - DNA, 102 bp, synthetic construct
  misc_feature 1..102: note = Description of Artificial Sequence: Synthetic polynucleotide
  source 1..102: mol_type = other DNA
aacatgaggatcacccatgtcgtctttgctctccccggacactctgctccttaaatgaaacacgggctcgtgcacggggccaacatgaggatcacccatgtc

SEQ ID NO: 75 - DNA, 72 bp, synthetic construct
  misc_feature 1..72: note = Description of Artificial Sequence: Synthetic oligonucleotide
  source 1..72: mol_type = other DNA
aacatgaggatcacccatgtccggactgagtgctcaaaatgattgtcgggcaacatgaggatcacccatgtc

SEQ ID NO: 76 - DNA, 82 bp, synthetic construct
  misc_feature 1..82: note = Description of Artificial Sequence: Synthetic oligonucleotide
  source 1..82: mol_type = other DNA
aacatgaggatcacccatgtctgctcagggcggactgagaaaattgtcgggcagcagcacgaacatgaggatcacccatgtc

SEQ ID NO: 77 - DNA, 18 bp, synthetic construct
  misc_feature 1..18: note = Description of Artificial Sequence: Synthetic oligonucleotide
  source 1..18: mol_type = other DNA
gcgcctccatcgaagtgt

SEQ ID NO: 78 - DNA, 16 bp, synthetic construct
  misc_feature 1..16: note = Description of Artificial Sequence: Synthetic oligonucleotide
  source 1..16: mol_type = other DNA
gccatctatcgatggg

SEQ ID NO: 79 - DNA, 16 bp, synthetic construct
  misc_feature 1..16: note = Description of Artificial Sequence: Synthetic oligonucleotide
  source 1..16: mol_type = other DNA
caaaccgagcggtgtc

SEQ ID NO: 80 - DNA, 16 bp, synthetic construct
  misc_feature 1..16: note = Description of Artificial Sequence: Synthetic oligonucleotide
  source 1..16: mol_type = other DNA
acaaaccgagcggtgt

SEQ ID NO: 81 - DNA, 16 bp, synthetic construct
  misc_feature 1..16: note = Description of Artificial Sequence: Synthetic oligonucleotide
  source 1..16: mol_type = other DNA
tacaaaccgagcggtg

SEQ ID NO: 82 - DNA, 16 bp, synthetic construct
  misc_feature 1..16: note = Description of Artificial Sequence: Synthetic oligonucleotide
  source 1..16: mol_type = other DNA
ttacaaaccgagcggt

SEQ ID NO: 83 - DNA, 17 bp, synthetic construct
  misc_feature 1..17: note = Description of Artificial Sequence: Synthetic oligonucleotide
  source 1..17: mol_type = other DNA
caaaccgagcggtgtct

SEQ ID NO: 84 - DNA, 17 bp, synthetic construct
  misc_feature 1..17: note = Description of Artificial Sequence: Synthetic oligonucleotide
  source 1..17: mol_type = other DNA
acaaaccgagcggtgtc

SEQ ID NO: 85 - DNA, 17 bp, synthetic construct
  misc_feature 1..17: note = Description of Artificial Sequence: Synthetic oligonucleotide
  source 1..17: mol_type = other DNA
tacaaaccgagcggtgt

SEQ ID NO: 86 - DNA, 17 bp, synthetic construct
  misc_feature 1..17: note = Description of Artificial Sequence: Synthetic oligonucleotide
  source 1..17: mol_type = other DNA
ttacaaaccgagcggtg

SEQ ID NO: 87 - DNA, 18 bp, synthetic construct
  misc_feature 1..18: note = Description of Artificial Sequence: Synthetic oligonucleotide
  source 1..18: mol_type = other DNA
caaaccgagcggtgtctg

SEQ ID NO: 88 - DNA, 18 bp, synthetic construct
  misc_feature 1..18: note = Description of Artificial Sequence: Synthetic oligonucleotide
  source 1..18: mol_type = other DNA
acaaaccgagcggtgtct

SEQ ID NO: 89 - DNA, 18 bp, synthetic construct
  misc_feature 1..18: note = Description of Artificial Sequence: Synthetic oligonucleotide
  source 1..18: mol_type = other DNA
tacaaaccgagcggtgtc

SEQ ID NO: 90 - DNA, 18 bp, synthetic construct
  misc_feature 1..18: note = Description of Artificial Sequence: Synthetic oligonucleotide
  source 1..18: mol_type = other DNA
ttacaaaccgagcggtgt

SEQ ID NO: 91 - DNA, 19 bp, synthetic construct
  misc_feature 1..19: note = Description of Artificial Sequence: Synthetic oligonucleotide
  source 1..19: mol_type = other DNA
caaaccgagcggtgtctgt

SEQ ID NO: 92 - DNA, 19 bp, synthetic construct
  misc_feature 1..19: note = Description of Artificial Sequence: Synthetic oligonucleotide
  source 1..19: mol_type = other DNA
acaaaccgagcggtgtctg

SEQ ID NO: 93 - DNA, 19 bp, synthetic construct
  misc_feature 1..19: note = Description of Artificial Sequence: Synthetic oligonucleotide
  source 1..19: mol_type = other DNA
tacaaaccgagcggtgtct

SEQ ID NO: 94 - DNA, 19 bp, synthetic construct
  misc_feature 1..19: note = Description of Artificial Sequence: Synthetic oligonucleotide
  source 1..19: mol_type = other DNA
ttacaaaccgagcggtgtc

SEQ ID NO: 95 - DNA, 20 bp, synthetic construct
  misc_feature 1..20: note = Description of Artificial Sequence: Synthetic oligonucleotide
  source 1..20: mol_type = other DNA
caaaccgagcggtgtctgtg

SEQ ID NO: 96 - DNA, 20 bp, synthetic construct
  misc_feature 1..20: note = Description of Artificial Sequence: Synthetic oligonucleotide
  source 1..20: mol_type = other DNA
acaaaccgagcggtgtctgt

SEQ ID NO: 97 - DNA, 20 bp, synthetic construct
  misc_feature 1..20: note = Description of Artificial Sequence: Synthetic oligonucleotide
  source 1..20: mol_type = other DNA
tacaaaccgagcggtgtctg

SEQ ID NO: 98 - DNA, 20 bp, synthetic construct
  misc_feature 1..20: note = Description of Artificial Sequence: Synthetic oligonucleotide
  source 1..20: mol_type = other DNA
ttacaaaccgagcggtgtct

SEQ ID NO: 99 - DNA, 21 bp, synthetic construct
  misc_feature 1..21: note = Description of Artificial Sequence: Synthetic oligonucleotide
  source 1..21: mol_type = other DNA
caaaccgagcggtgtctgtga

SEQ ID NO: 100 - DNA, 21 bp, synthetic construct
  misc_feature 1..21: note = Description of Artificial Sequence: Synthetic oligonucleotide
  source 1..21: mol_type = other DNA
acaaaccgagcggtgtctgtg

SEQ ID NO: 101 - DNA, 21 bp, synthetic construct
  misc_feature 1..21: note = Description of Artificial Sequence: Synthetic oligonucleotide
  source 1..21: mol_type = other DNA
tacaaaccgagcggtgtctgt

SEQ ID NO: 102 - DNA, 21 bp, synthetic construct
  misc_feature 1..21: note = Description of Artificial Sequence: Synthetic oligonucleotide
  source 1..21: mol_type = other DNA
ttacaaaccgagcggtgtctg

SEQ ID NO: 103 - DNA, 66 bp, unidentified
  misc_feature 1..66: note = Description of Unknown: target sequence
  source 1..66: mol_type = other DNA
cacttgggtgtgaatgaaagtctcacagacaccgctcagtttgtaaaacttttcttccttccaaag

SEQ ID NO: 104 - DNA, 62 bp, synthetic construct
  misc_feature 1..62: note = Description of Artificial Sequence: Synthetic oligonucleotide
  source 1..62: mol_type = other DNA
aacatgaggatcacccatgtccaaaccgagcggtgtctgtgaacatgaggatcacccatgtc

SEQ ID NO: 105 - DNA, 62 bp, synthetic construct
  misc_feature 1..62: note = Description of Artificial Sequence: Synthetic oligonucleotide
  source 1..62: mol_type = other DNA
aacatgaggatcacccatgtctacaaaccgagcggtgtctgaacatgaggatcacccatgtc

SEQ ID NO: 106 - DNA, 62 bp, synthetic construct
  misc_feature 1..62: note = Description of Artificial Sequence: Synthetic oligonucleotide
  source 1..62: mol_type = other DNA
aacatgaggatcacccatgtctttacaaaccgagcggtgtcaacatgaggatcacccatgtc

SEQ ID NO: 107 - DNA, 66 bp, synthetic construct
  misc_feature 1..66: note = Description of Artificial Sequence: Synthetic oligonucleotide
  source 1..66: mol_type = other DNA
aacatgaggatcacccatgtccaaaccgagcggtgtctgtgagacaacatgaggatcacccatgtc

SEQ ID NO: 108 - DNA, 58 bp, synthetic construct
  misc_feature 1..58: note = Description of Artificial Sequence: Synthetic oligonucleotide
  source 1..58: mol_type = other DNA
aacatgaggatcacccatgtccaaaccgagcggtgtcaacatgaggatcacccatgtc

SEQ ID NO: 109 - DNA, 82 bp, synthetic construct
  misc_feature 1..82: note = Description of Artificial Sequence: Synthetic oligonucleotide
  source 1..82: mol_type = other DNA
aagaaaagttaacatgaggatcacccatgtccaaaccgagcggtgtctgtgaacatgaggatcacccatgtcctttcattca

SEQ ID NO: 110 - DNA, 102 bp, synthetic construct
  misc_feature 1..102: note = Description of Artificial Sequence: Synthetic polynucleotide
  source 1..102: mol_type = other DNA
ctttggaaggaagaaaagttaacatgaggatcacccatgtccaaaccgagcggtgtctgtgaacatgaggatcacccatgtcctttcattcacacccaagtg

SEQ ID NO: 111 - DNA, 31 bp, synthetic construct
  misc_feature 1..31: note = Description of Artificial Sequence: Synthetic oligonucleotide
  source 1..31: mol_type = other DNA
ttgggaaatccagctagcggcagtattctgt

SEQ ID NO: 112 - DNA, 31 bp, unidentified
  misc_feature 1..31: note = Description of Unknown: target sequence
  source 1..31: mol_type = other DNA
gggcgatgccacctaaggcaagctgaccctg

SEQ ID NO: 113 - DNA, 19 bp, synthetic construct
  misc_feature 1..19: note = Description of Artificial Sequence: Synthetic oligonucleotide
  source 1..19: mol_type = other DNA
gccctaggtggcatcgccc

SEQ ID NO: 114 - DNA, 19 bp, synthetic construct
  misc_feature 1..19: note = Description of Artificial Sequence: Synthetic oligonucleotide
  source 1..19: mol_type = other DNA
cagggtcagcttgccctag

SEQ ID NO: 115 - DNA, 19 bp, synthetic construct
  misc_feature 1..19: note = Description of Artificial Sequence: Synthetic oligonucleotide
  source 1..19: mol_type = other DNA
gccccaggtggcatcgccc

SEQ ID NO: 116 - DNA, 19 bp, synthetic construct
  misc_feature 1..19: note = Description of Artificial Sequence: Synthetic oligonucleotide
  source 1..19: mol_type = other DNA
agggtcagcttgccccagg

SEQ ID NO: 117 - DNA, 14 bp, synthetic construct
  misc_feature 1..14: note = Description of Artificial Sequence: Synthetic oligonucleotide
  source 1..14: mol_type = other DNA
agcaataaaatggc

SEQ ID NO: 118 - DNA, 14 bp, synthetic construct
  misc_feature 1..14: note = Description of Artificial Sequence: Synthetic oligonucleotide
  source 1..14: mol_type = other DNA
agcaataaaatggc

SEQ ID NO: 119 - DNA, 34 bp, Mus sp.
  source 1..34: mol_type = other DNA
gagcaataaaatggcttcaactatctgagtgaca

SEQ ID NO: 120 - DNA, 34 bp, Mus sp.; identical to SEQ ID NO: 119
  source 1..34: mol_type = other DNA

SEQ ID NO: 121 - DNA, 34 bp, synthetic construct
  misc_feature 1..34: note = Description of Artificial Sequence: Synthetic oligonucleotide
  source 1..34: mol_type = other DNA
gagccataaaatggcttcaactatctgagtgaca

SEQ ID NO: 122 - DNA, 34 bp, Mus sp.; identical to SEQ ID NO: 119
  source 1..34: mol_type = other DNA

SEQ ID NO: 123 - DNA, 34 bp, synthetic construct
  misc_feature 1..34: note = Description of Artificial Sequence: Synthetic oligonucleotide
  source 1..34: mol_type = other DNA
gagcaatggaatggcttcaactatctgagtgaca

SEQ ID NO: 124 - DNA, 34 bp, synthetic construct; identical to SEQ ID NO: 121
  misc_feature 1..34: note = Description of Artificial Sequence: Synthetic oligonucleotide
  source 1..34: mol_type = other DNA

SEQ ID NO: 125 - DNA, 34 bp, Mus sp.; identical to SEQ ID NO: 119
  source 1..34: mol_type = other DNA

SEQ ID NO: 126 - DNA, 34 bp, synthetic construct; identical to SEQ ID NO: 123
  misc_feature 1..34: note = Description of Artificial Sequence: Synthetic oligonucleotide
  source 1..34: mol_type = other DNA

SEQ ID NO: 127 - DNA, 34 bp, Mus sp.; identical to SEQ ID NO: 119
  source 1..34: mol_type = other DNA

SEQ ID NO: 128 - DNA, 34 bp, synthetic construct; identical to SEQ ID NO: 123
  misc_feature 1..34: note = Description of Artificial Sequence: Synthetic oligonucleotide
  source 1..34: mol_type = other DNA

SEQ ID NO: 129 - DNA, 34 bp, synthetic construct
  misc_feature 1..34: note = Description of Artificial Sequence: Synthetic oligonucleotide
  source 1..34: mol_type = other DNA
gagcaatgaaatggcttcaactatctgagtgaca

SEQ ID NO: 130 - DNA, 34 bp, synthetic construct
  misc_feature 1..34: note = Description of Artificial Sequence: Synthetic oligonucleotide
  source 1..34: mol_type = other DNA
gagcagtggaatggcttcaactatctgagtgaca

SEQ ID NO: 131 - DNA, 13 bp, synthetic construct
  misc_feature 1..13: note = Description of Artificial Sequence: Synthetic oligonucleotide
  modified_base 12: mod_base = OTHER; note = a, c, t, g, unknown or other
  source 1..13: mol_type = other DNA
ccgctcagtttnt

SEQ ID NO: 132 - DNA, 13 bp, synthetic construct
  misc_feature 1..13: note = Description of Artificial Sequence: Synthetic oligonucleotide
  modified_base 7..8: mod_base = OTHER; note = a, c, t, g, unknown or other
  modified_base 12: mod_base = OTHER; note = a, c, t, g, unknown or other
  source 1..13: mol_type = other DNA
ccgctcnntttnt

SEQ ID NO: 133 - DNA, 28 bp, Mus sp.
  source 1..28: mol_type = other DNA
agacaccgctcatgtcttatctagcatg

SEQ ID NO: 134 - DNA, 28 bp, Mus sp.
  source 1..28: mol_type = other DNA
agacaccgctcatgtcttatctagcatg

SEQ ID NO: 135 - DNA, 28 bp, synthetic construct
  misc_feature 1..28: note = Description of Artificial Sequence: Synthetic oligonucleotide
  source 1..28: mol_type = other DNA
agacaccgctcgtgtcttatctagcatg

SEQ ID NO: 136 - DNA, 28 bp, Mus sp.
  source 1..28: mol_type = other DNA
agacaccgctcatgtcttatctagcatg

SEQ ID NO: 137 - DNA, 28 bp, synthetic construct
  misc_feature 1..28: note = Description of Artificial Sequence: Synthetic oligonucleotide
  source 1..28: mol_type = other DNA
agacaccgctcgtgtcttatctagcatg

SEQ ID NO: 138 - DNA, 28 bp, Mus sp.
  source 1..28: mol_type = other DNA
agacaccgctcatgtcttatctagcatg

SEQ ID NO: 139 - DNA, 28 bp, synthetic construct
  misc_feature 1..28: note = Description of Artificial Sequence: Synthetic oligonucleotide
  source 1..28: mol_type = other DNA
agacaccgctcgtgtcttatctagcatg

SEQ ID NO: 140 - protein, 429 aa, unidentified
  REGION 1..429: note = Description of Unknown: ADAR1 catalytic domain sequence
KAERMGFTEVTPVTGASLRRTMLLLSRSPEAQPKTLPLTGSTFHDQIAMLSHRCFNTLTNSFQPSLLGRKILAAIIMKKDSEDMGVVVSLGTGNRCVKGDSLSLKGETVNDCHAEIISRRGFIRFLYSELMKYNSQTAKDSIFEPAKGGEKLQIKKTVSFHLYISTAPCGDGALFDKSCSDRAMESTESRHYPVFENPKQGKLRTKVENGEGTIPVESSDIVPTWDGIRLGERLRTMSCSDKILRWNVLGLQGALLTHFLQPIYLKSVTLGYLFSQGHLTRAICCRVTRDGSAFEDGLRHPFIVNHPKVGRVSIYDSKRQSGKTKETSVNWCLADGYDLEILDGTRGTVDGPRNELSRVSKKNIFLLFKKLCSFRYRRDLLRLSYGEAKKAARDYETAKNYFKKGLKDMGYGNWISKPQEEKNFYLCPV

SEQ ID NO: 141 - protein, 385 aa, unidentified
  REGION 1..385: note = Description of Unknown: ADAR2 catalytic domain sequence
QLHLPQVLADAVSRLVLGKFGDLTDNFSSPHARRKVLAGVVMTTGTDVKDAKVISVSTGTKCINGEYMSDRGLALNDCHAEIISRRSLLRFLYTQLELYLNNKDDQKRSIFQKSERGGFRLKENVQFHLYISTSPCGDARIFSPHEPILEEPADRHPNRKARGQLRTKIESGEGTIPVRSNASIQTWDGVLQGERLLTMSCSDKIARWNVVGIQGSLLSIFVEPIYFSSIILGSLYHGDHLSRAMYQRISNIEDLPPLYTLNKPLLSGISNAEARQPGKAPNFSVNWTVGDSAIEVINATTGKDELGRASRLCKHALYCRWMRVHGKVPSHLLRSKITKPNVYHESKLAAKEYQAAKARLFTAFIKAGLGAWVEKPTEQDQFSLT

SEQ ID NO: 142 - protein, 298 aa, unidentified
  REGION 1..298: note = Description of Unknown: ADAR dsRBD sequence
MDIEDEENMSSSSTDVKENRNLDNVSPKDGSTPGPGEGSQLSNGGGGGPGRKRPLEEGSNGHSKYRLKKRRKTPGPVLPKNALMQLNEIKPGLQYTLLSQTGPVHAPLFVMSVEVNGQVFEGSGPTKKKAKLHAAEKALRSFVQFPNASEAHLAMGRTLSVNTDFTSDQADFPDTLFNGFETPDKAEPPFYVGSNGDDSFSSSGDLSLSASPVPASLAQPPLPVLPPFPPPSGKNPVMILNELRPGLKYDFLSESGESHAKSFVMSVVVDGQFFEGSGRNKKLAKARAAQSALAAIFN

SEQ ID NO: 143 - protein, 564 aa, synthetic construct
  REGION 1..564: note = Description of Artificial Sequence: Synthetic polypeptide
MLRSFVQFPNASEAHLAMGRTLSVNTDFTSDQADFPDTLFNGFETPDKAEPPFYVGSNGDDSFSSSGDLSLSASPVPASLAQPPLPVLPPFPPPSGKNPVMILNELRPGLKYDFLSESGESHAKSFVMSVVVDGQFFEGSGRNKKLAKARAAQSALAAIFNLHLDQTPSRQPIPSEGLQLHLPQVLADAVSRLVLGKFGDLTDNFSSPHARRKVLAGVVMTTGTDVKDAKVISVSTGTKCINGEYMSDRGLALNDCHAEIISRRSLLRFLYTQLELYLNNKDDQKRSIFQKSERGGFRLKENVQFHLYISTSPCGDARIFSPHEPILEEPADRHPNRKARGQLRTKIESGEGTIPVRSNASIQTWDGVLQGERLLTMSCSDKIARWNVVGIQGSLLSIFVEPIYFSSIILGSLYHGDHLSRAMYQRISNIEDLPPLYTLNKPLLSGISNAEARQPGKAPNFSVNWTVGDSAIEVINATTGKDELGRASRLCKHALYCRWMRVHGKVPSHLLRSKITKPNVYHESKLAAKEYQAAKARLFTAFIKAGLGAWVEKPTEQDQFSLTP

SEQ ID NO: 144 - DNA, 36 bp, Mus sp.
  source 1..36: mol_type = other DNA
ctcacagacaccgctcggtttgtaaaacttttcttc

SEQ ID NO: 145 - DNA, 36 bp, synthetic construct
  misc_feature 1..36: note = Description of Artificial Sequence: Synthetic oligonucleotide
  source 1..36: mol_type = other DNA
ctcacagacaccgctcagtttgtaaaacttttcttc

SEQ ID NO: 146 - DNA, 36 bp, synthetic construct; identical to SEQ ID NO: 145
  misc_feature 1..36: note = Description of Artificial Sequence: Synthetic oligonucleotide
  source 1..36: mol_type = other DNA

SEQ ID NO: 147 - DNA, 36 bp, synthetic construct
  misc_feature 1..36: note = Description of Artificial Sequence: Synthetic oligonucleotide
  source 1..36: mol_type = other DNA
ctcacagacaccgctcatgtcttatctagcatgaca

SEQ ID NO: 148 - DNA, 36 bp, synthetic construct
  misc_feature 1..36: note = Description of Artificial Sequence: Synthetic oligonucleotide
  source 1..36: mol_type = other DNA
ctcacagacaccgctcgtgtcttatctagcatgaca

SEQ ID NO: 149 - DNA, 16 bp, synthetic construct
  misc_feature 1..16: note = Description of Artificial Sequence: Synthetic primer
  source 1..16: mol_type = other DNA
cggcctcagtgagcga

SEQ ID NO: 150 - DNA, 21 bp, synthetic construct
  misc_feature 1..21: note = Description of Artificial Sequence: Synthetic primer
  source 1..21: mol_type = other DNA
ggaacccctagtgatggagtt

SEQ ID NO: 151 - DNA, 51 bp, Homo sapiens
  source 1..51: mol_type = other DNA
agcggcagtattctgtacagtagacacaagaattatgtacgccttttatca

SEQ ID NO: 152 - DNA, 66 bp, synthetic construct; identical to SEQ ID NO: 2
  misc_feature 1..66: note = Description of Artificial Sequence: Synthetic oligonucleotide
  modified_base 46..51: mod_base = OTHER; note = a, c, t, g, unknown or other
  modified_base 53..66: mod_base = OTHER; note = a, c, t, g, unknown or other
  source 1..66: mol_type = other DNA

SEQ ID NO: 153 - DNA, 76 bp, synthetic construct
  misc_feature 1..76: note = Description of Artificial Sequence: Synthetic oligonucleotide
  modified_base 56..61: mod_base = OTHER; note = a, c, t, g, unknown or other
  modified_base 63..76: mod_base = OTHER; note = a, c, t, g, unknown or other
  source 1..76: mol_type = other DNA
ggtgtcgagaagaggagaacaatatgctaaatgttgttctcgtctcctcgacaccnnnnnncnnnnnnnnnnnnnn

SEQ ID NO: 154 - DNA, 65 bp, synthetic construct
  misc_feature 1..65: note = Description of Artificial Sequence: Synthetic oligonucleotide
  source 1..65: mol_type = other DNA
gtggaagaggagaacaatatgctaaatgttgttctcgtctcccactgccgccagctggatttccc

SEQ ID NO: 155 - DNA, 75 bp, synthetic construct
  misc_feature 1..75: note = Description of Artificial Sequence: Synthetic oligonucleotide
  source 1..75: mol_type = other DNA
ggtgtcgagaagaggagaacaatatgctaaatgttgttctcgtctcctcgacacctgccgccagctggatttccc

SEQ ID NO: 156 - DNA, 65 bp, synthetic construct
  misc_feature 1..65: note = Description of Artificial Sequence: Synthetic oligonucleotide
  source 1..65: mol_type = other DNA
gtggaagaggagaacaatatgctaaatgttgttctcgtctcccacctcctccacccgaccccggg

SEQ ID NO: 157 - DNA, 75 bp, synthetic construct
  misc_feature 1..75: note = Description of Artificial Sequence: Synthetic oligonucleotide
  source 1..75: mol_type = other DNA
ggtgtcgagaagaggagaacaatatgctaaatgttgttctcgtctcctcgacaccctcctccacccgaccccggg

SEQ ID NO: 158 - DNA, 65 bp, synthetic construct
  misc_feature 1..65: note = Description of Artificial Sequence: Synthetic oligonucleotide
  source 1..65: mol_type = other DNA
gtggaatagtataacaatatgctaaatgttgttatagtatcccacgagccccaaaattaaataga

SEQ ID NO: 159 - DNA, 65 bp, synthetic construct
  misc_feature 1..65: note = Description of Artificial Sequence: Synthetic oligonucleotide
  source 1..65: mol_type = other DNA
gtggaatagtataacaatatgctaaatgttgttatagtatcccacttacccgaaattttcgaagt

SEQ ID NO: 160 - DNA, 62 bp, synthetic construct
  misc_feature 1..62: note = Description of Artificial Sequence: Synthetic oligonucleotide
  source 1..62: mol_type = other DNA
aacatgaggatcacccatgtcgagccccaaaattaaatagaaacatgaggatcacccatgtc

SEQ ID NO: 161 - DNA, 62 bp, synthetic construct
  misc_feature 1..62: note = Description of Artificial Sequence: Synthetic oligonucleotide
  source 1..62: mol_type = other DNA
aacatgaggatcacccatgtcttacccgaaattttcgaagtaacatgaggatcacccatgtc

SEQ ID NO: 162 - DNA, 62 bp, synthetic construct
  misc_feature 1..62: note = Description of Artificial Sequence: Synthetic oligonucleotide
  source 1..62: mol_type = other DNA
aacatgaggatcacccatgtcccattccattgctctttcaaaacatgaggatcacccatgtc

SEQ ID NO: 163 - DNA, 65 bp, synthetic construct
  misc_feature 1..65: note = Description of Artificial Sequence: Synthetic oligonucleotide
  source 1..65: mol_type = other DNA
gtggaatagtataacaatatgctaaatgttgttatagtatcccacactgcccacagatgaacaag

SEQ ID NO: 164 - DNA, 65 bp, synthetic construct
  misc_feature 1..65: note = Description of Artificial Sequence: Synthetic oligonucleotide
  source 1..65: mol_type = other DNA
gtggaatagtataacaatatgctaaatgttgttatagtatcccactgtacccgaaggagagaata

SEQ ID NO: 165 - DNA, 65 bp, synthetic construct
  misc_feature 1..65: note = Description of Artificial Sequence: Synthetic oligonucleotide
  source 1..65: mol_type = other DNA
gtggaatagtataacaatatgctaaatgttgttatagtatcccacaaagtccgaggaggaaaaag

SEQ ID NO: 166 - DNA, 65 bp, synthetic construct
  misc_feature 1..65: note = Description of Artificial Sequence: Synthetic oligonucleotide
  source 1..65: mol_type = other DNA
gtggaatagtataacaatatgctaaatgttgttatagtatcccacaatacccgtaggattaaatc

SEQ ID NO: 167 - DNA, 65 bp, synthetic construct
  misc_feature 1..65: note = Description of Artificial Sequence: Synthetic oligonucleotide
  source 1..65: mol_type = other DNA
gtggaatagtataacaatatgctaaatgttgttatagtatcccacaagttccggaaaacaaacaa

SEQ ID NO: 168 - DNA, 62 bp, synthetic construct
  misc_feature 1..62: note = Description of Artificial Sequence: Synthetic oligonucleotide
  source 1..62: mol_type = other DNA
aacatgaggatcacccatgtcactgcccacagatgaacaagaacatgaggatcacccatgtc

SEQ ID NO: 169 - DNA, 62 bp, synthetic construct
  misc_feature 1..62: note = Description of Artificial Sequence: Synthetic oligonucleotide
  source 1..62: mol_type = other DNA
aacatgaggatcacccatgtctgtacccgaaggagagaataaacatgaggatcacccatgtc

SEQ ID NO: 170 - DNA, 62 bp, synthetic construct
  misc_feature 1..62: note = Description of Artificial Sequence: Synthetic oligonucleotide
  source 1..62: mol_type = other DNA
aacatgaggatcacccatgtcaaagtccgaggaggaaaaagaacatgaggatcacccatgtc

SEQ ID NO: 171 - DNA, 62 bp, synthetic construct
  misc_feature 1..62: note = Description of Artificial Sequence: Synthetic oligonucleotide
  source 1..62: mol_type = other DNA
aacatgaggatcacccatgtcaatacccgtaggattaaatcaacatgaggatcacccatgtc

SEQ ID NO: 172 - DNA, 62 bp, synthetic construct
  misc_feature 1..62: note = Description of Artificial Sequence: Synthetic oligonucleotide
  source 1..62: mol_type = other DNA
aacatgaggatcacccatgtcaagttccggaaaacaaacaaaacatgaggatcacccatgtc

SEQ ID NO: 173 - DNA, 63 bp, synthetic construct
  misc_feature 1..63: note = Description of Artificial Sequence: Synthetic oligonucleotide
  modified_base 13..22: mod_base = OTHER; note = a, c, t, g, unknown or other
  modified_base 44..63: mod_base = OTHER; note = a, c, t, g, unknown or other
  source 1..63: mol_type = other DNA
acatatatgatannnnnnnnnnaacatgaggatcacccatgtcnnnnnnnnnnnnnnnnnnnn

SEQ ID NO: 174 - DNA, 66 bp, synthetic construct
  misc_feature 1..66: note = Description of Artificial Sequence: Synthetic oligonucleotide
  modified_base 1..20: mod_base = OTHER; note = a, c, t, g, unknown or other
  modified_base 42..51: mod_base = OTHER; note = a, c, t, g, unknown or other
  source 1..66: mol_type = other DNA
nnnnnnnnnnnnnnnnnnnnaacatgaggatcacccatgtcnnnnnnnnnnttgatcagtatatta

SEQ ID NO: 175 - DNA, 30 bp, synthetic construct
  misc_feature 1..30: note = Description of Artificial Sequence: Synthetic oligonucleotide
  source 1..30: mol_type = other DNA
acatatatgatacaatttgatcagtatatt

SEQ ID NO: 176 - DNA, 30 bp, synthetic construct; identical to SEQ ID NO: 175
  misc_feature 1..30: note = Description of Artificial Sequence: Synthetic oligonucleotide
  source 1..30: mol_type = other DNA

SEQ ID NO: 177 - DNA, 21 bp, synthetic construct
  misc_feature 1..21: note = Description of Artificial Sequence: Synthetic oligonucleotide
  source 1..21: mol_type = other DNA
aacatgaggatcacccatgtc

SEQ ID NO: 178 - DNA, 120 bp, synthetic construct
  misc_feature 1..120: note = Description of Artificial Sequence: Synthetic polynucleotide
  source 1..120: mol_type = other DNA
gtggaatagtataacaatatgctaaatgttgttatagtatcccactgccgccagctggatttcccaattctgagtgtggaatagtataacaatatgctaaatgttgttatagtatcccac

SEQ ID NO: 179 - DNA, 130 bp, synthetic construct
  misc_feature 1..130: note = Description of Artificial Sequence: Synthetic polynucleotide
  source 1..130: mol_type = other DNA
gtggaatagtataacaatatgctaaatgttgttatagtatcccactgccgccagctggatttcccaattctgagtaacactctgcgtggaatagtataacaatatgctaaatgttgttatagtatcccac

SEQ ID NO: 180 - DNA, 150 bp, synthetic construct
  misc_feature 1..150: note = Description of Artificial Sequence: Synthetic polynucleotide
  source 1..150: mol_type = other DNA
gtggaatagtataacaatatgctaaatgttgttatagtatcccactgccgccagctggatttcccaattctgagtaacactctgcaatccaaacagggttcaaccgtggaatagtataacaatatgctaaatgttgttatagtatcccac

SEQ ID NO: 181 - DNA, 170 bp, synthetic construct
  misc_feature 1..170: note = Description of Artificial Sequence: Synthetic polynucleotide
  source 1..170: mol_type = other DNA
gtggaatagtataacaatatgctaaatgttgttatagtatcccactgccgccagctggatttcccaattctgagtaacactctgcaatccaaacagggttcaaccctccaccttacaggcctgcagtggaatagtataacaatatgctaaatgttgttatagtatcccac

SEQ ID NO: 182 - DNA, 190 bp, synthetic construct
  misc_feature 1..190: note = Description of Artificial Sequence: Synthetic polynucleotide
  source 1..190: mol_type = other DNA
gtggaatagtataacaatatgctaaatgttgttatagtatcccactgccgccagctggatttcccaattctgagtaacactctgcaatccaaacagggttcaaccctccaccttacaggcctgcattacaggacttaaacacatagtggaatagtataacaatatgctaaatgttgttatagtatcccac

SEQ ID NO: 183 - DNA, 210 bp, synthetic construct
  misc_feature 1..210: note = Description of Artificial Sequence: Synthetic polynucleotide
  source 1..210: mol_type = other DNA
gtggaatagtataacaatatgctaaatgttgttatagtatcccactgccgccagctggatttcccaattctgagtaacactctgcaatccaaacagggttcaaccctccaccttacaggcctgcattacaggacttaaacacataatccaagaatttcttacactgtggaatagtataacaatatgctaaatgttgttatagtatcccac

SEQ ID NO: 184 - DNA, 110 bp, synthetic construct
  misc_feature 1..110: note = Description of Artificial Sequence: Synthetic polynucleotide
  source 1..110: mol_type = other DNA
gtggaatagtataacaatatgctaaatgttgttatagtatcccacatactgccgccagctggattgtggaatagtataacaatatgctaaatgttgttatagtatcccac

SEQ ID NO: 185 - DNA, 130 bp, synthetic construct
  misc_feature 1..130: note = Description of Artificial Sequence: Synthetic polynucleotide
  source 1..130: mol_type = other DNA
gtggaatagtataacaatatgctaaatgttgttatagtatcccacactgtacagaatactgccgccagctggatttcccaattctgtggaatagtataacaatatgctaaatgttgttatagtatcccac

SEQ ID NO: 186 - DNA, 150 bp, synthetic construct
  misc_feature 1..150: note = Description of Artificial Sequence: Synthetic polynucleotide
  source 1..150: mol_type = other DNA
gtggaatagtataacaatatgctaaatgttgttatagtatcccactcttgtgtctactgtacagaatactgccgccagctggatttcccaattctgagtaacactgtggaatagtataacaatatgctaaatgttgttatagtatcccac

SEQ ID NO: 187 - DNA, 170 bp, synthetic construct
  misc_feature 1..170: note = Description of Artificial Sequence: Synthetic polynucleotide
  source 1..170: mol_type = other DNA
gtggaatagtataacaatatgctaaatgttgttatagtatcccaccgtacataattcttgtgtctactgtacagaatactgccgccagctggatttcccaattctgagtaacactctgcaatccagtggaatagtataacaatatgctaaatgttgttatagtatcccac

SEQ ID NO: 188 - DNA, 190 bp, synthetic construct
  misc_feature 1..190: note = Description of Artificial Sequence: Synthetic polynucleotide
  source 1..190: mol_type = other DNA
gtggaatagtataacaatatgctaaatgttgttatagtatcccactgataaaaggcgtacataattcttgtgtctactgtacagaatactgccgccagctggatttcccaattctgagtaacactctgcaatccaaacagggttcgtggaatagtataacaatatgctaaatgttgttatagtatcccac

SEQ ID NO: 189 - DNA, 210 bp, synthetic construct
  misc_feature 1..210: note = Description of Artificial Sequence: Synthetic polynucleotide
  source 1..210: mol_type = other DNA
gtggaatagtataacaatatgctaaatgttgttatagtatcccaccttaagtctttgataaaaggcgtacataattcttgtgtctactgtacagaatactgccgccagctggatttcccaattctgagtaacactctgcaatccaaacagggttcaaccctccacgtggaatagtataacaatatgctaaatgttgttatagtatcccac

SEQ ID NO: 190 - DNA, 120 bp, synthetic construct
  misc_feature 1..120: note = Description of Artificial Sequence: Synthetic polynucleotide
  source 1..120: mol_type = other DNA
gtggaagaggagaacaataggctaaacgttgttctcgtctcccactgccgccagctggatttcccaattctgagtgtggaagaggagaacaataggctaaacgttgttctcgtctcccac

SEQ ID NO: 191 - DNA, 130 bp, synthetic construct
  misc_feature 1..130: note = Description of Artificial Sequence: Synthetic polynucleotide
  source 1..130: mol_type = other DNA
gtggaagaggagaacaataggctaaacgttgttctcgtctcccactgccgccagctggatttcccaattctgagtaacactctgcgtggaagaggagaacaataggctaaacgttgttctcgtctcccac

SEQ ID NO: 192 - DNA, 150 bp, synthetic construct
  misc_feature 1..150: note = Description of Artificial Sequence: Synthetic polynucleotide
  source 1..150: mol_type = other DNA
gtggaagaggagaacaataggctaaacgttgttctcgtctcccactgccgccagctggatttcccaattctgagtaacactctgcaatccaaacagggttcaaccgtggaagaggagaacaataggctaaacgttgttctcgtctcccac

SEQ ID NO: 193 - DNA, 170 bp, synthetic construct
  misc_feature 1..170: note = Description of Artificial Sequence: Synthetic polynucleotide
  source 1..170: mol_type = other DNA
gtggaagaggagaacaataggctaaacgttgttctcgtctcccactgccgccagctggatttcccaattctgagtaacactctgcaatccaaacagggttcaaccctccaccttacaggcctgcagtggaagaggagaacaataggctaaacgttgttctcgtctcccac

SEQ ID NO: 194 - DNA, 190 bp, synthetic construct
  misc_feature 1..190: note = Description of Artificial Sequence: Synthetic polynucleotide
  source 1..190: mol_type = other DNA
gtggaagaggagaacaataggctaaacgttgttctcgtctcccactgccgccagctggatttcccaattctgagtaacactctgcaatccaaacagggttcaaccctccaccttacaggcctgcattacaggacttaaacacatagtggaagaggagaacaataggctaaacgttgttctcgtctcccac

SEQ ID NO: 195 - DNA, 210 bp, synthetic construct
  misc_feature 1..210: note = Description of Artificial Sequence: Synthetic polynucleotide
  source 1..210: mol_type = other DNA
gtggaagaggagaacaataggctaaacgttgttctcgtctcccactgccgccagctggatttcccaattctgagtaacactctgcaatccaaacagggttcaaccctccaccttacaggcctgcattacaggacttaaacacataatccaagaatttcttacactgtggaagaggagaacaataggctaaacgttgttctcgtctcccac

SEQ ID NO: 196 - DNA, 110 bp, synthetic construct
  misc_feature 1..110: note = Description of Artificial Sequence: Synthetic polynucleotide
  source 1..110: mol_type = other DNA
gtggaagaggagaacaataggctaaacgttgttctcgtctcccacatactgccgccagctggattgtggaagaggagaacaataggctaaacgttgttctcgtctcccac

SEQ ID NO: 197 - DNA, 130 bp, synthetic construct
  misc_feature 1..130: note = Description of Artificial Sequence: Synthetic polynucleotide
  source 1..130: mol_type = other DNA
gtggaagaggagaacaataggctaaacgttgttctcgtctcccacactgtacagaatactgccgccagctggatttcccaattctgtggaagaggagaacaataggctaaacgttgttctcgtctcccac

SEQ ID NO: 198 - DNA, 150 bp, synthetic construct
  misc_feature 1..150: note = Description of Artificial Sequence: Synthetic polynucleotide
  source 1..150: mol_type = other DNA
gtggaagaggagaacaataggctaaacgttgttctcgtctcccactcttgtgtctactgtacagaatactgccgccagctggatttcccaattctgagtaacactgtggaagaggagaacaataggctaaacgttgttctcgtctcccac

SEQ ID NO: 199 - DNA, 170 bp, synthetic construct
  misc_feature 1..170: note = Description of Artificial Sequence: Synthetic polynucleotide
  source 1..170: mol_type = other DNA
gtggaagaggagaacaataggctaaacgttgttctcgtctcccaccgtacataattcttgtgtctactgtacagaatactgccgccagctggatttcccaattctgagtaacactctgcaatccagtggaagaggagaacaataggctaaacgttgttctcgtctcccac

SEQ ID NO: 200 - DNA, 190 bp, synthetic construct
  misc_feature 1..190: note = Description of Artificial Sequence: Synthetic polynucleotide
  source 1..190: mol_type = other DNA
gtggaagaggagaacaataggctaaacgttgttctcgtctcccactgataaaaggcgtacataattcttgtgtctactgtacagaatactgccgccagctggatttcccaattctgagtaacactctgcaatccaaacagggttcgtggaagaggagaacaataggctaaacgttgttctcgtctcccac

SEQ ID NO: 201 - DNA, 210 bp, synthetic construct
  misc_feature 1..210: note = Description of Artificial Sequence: Synthetic polynucleotide
  source 1..210: mol_type = other DNA
gtggaagaggagaacaataggctaaacgttgttctcgtctcccaccttaagtctttgataaaaggcgtacataattcttgtgtctactgtacagaatactgccgccagctggatttcccaattctgagtaacactctgcaatccaaacagggttcaaccctccacgtggaagaggagaacaataggctaaacgttgttctcgtctcccac

SEQ ID NO: 202 - DNA, 20 bp, synthetic construct
  misc_feature 1..20: note = Description of Artificial Sequence: Synthetic oligonucleotide
  source 1..20: mol_type = other DNA
acaaaccgagcggtgtctgt

SEQ ID NO: 203 - DNA, 20 bp, synthetic construct
  misc_feature 1..20: note = Description of Artificial Sequence: Synthetic oligonucleotide
  source 1..20: mol_type = other DNA
gccattccattgctctttca

SEQ ID NO: 204 - DNA, 20 bp, synthetic construct
  misc_feature 1..20: note = Description of Artificial Sequence: Synthetic oligonucleotide
  source 1..20: mol_type = other DNA
tgccgccagctggatttccc

SEQ ID NO: 205 - DNA, 20 bp, synthetic construct
  misc_feature 1..20: note = Description of Artificial Sequence: Synthetic oligonucleotide
  source 1..20: mol_type = other DNA
ctgtaccagccagtcaatta

SEQ ID NO: 206 - DNA, 20 bp, synthetic construct
  misc_feature 1..20: note = Description of Artificial Sequence: Synthetic oligonucleotide
  source 1..20: mol_type = other DNA
cttctccacagcccgaagca

SEQ ID NO: 207 - DNA, 20 bp, synthetic construct
  misc_feature 1..20: note = Description of Artificial Sequence: Synthetic oligonucleotide
  source 1..20: mol_type = other DNA
ctcctccacccgaccccggg

SEQ ID NO: 208 - DNA, 20 bp, synthetic construct
  misc_feature 1..20: note = Description of Artificial Sequence: Synthetic oligonucleotide
  source 1..20: mol_type = other DNA
gggtgccaagcagttggtgg

SEQ ID NO: 209 - DNA, 20 bp, synthetic construct
  misc_feature 1..20: note = Description of Artificial Sequence: Synthetic oligonucleotide
  source 1..20: mol_type = other DNA
cttgtccaccttgatgccca

SEQ ID NO: 210 - DNA, 20 bp, synthetic construct
  misc_feature 1..20: note = Description of Artificial Sequence: Synthetic oligonucleotide
  source 1..20: mol_type = other DNA
ttcatccaatggctggttat

SEQ ID NO: 211 - DNA, 20 bp, synthetic construct
  misc_feature 1..20: note = Description of Artificial Sequence: Synthetic oligonucleotide
  source 1..20: mol_type = other DNA
caaggccaagggctcgccag

SEQ ID NO: 212 - DNA, 20 bp, synthetic construct
  misc_feature 1..20: note = Description of Artificial Sequence: Synthetic oligonucleotide
  source 1..20: mol_type = other DNA
tccaaccaccacaagtttat

SEQ ID NO: 213 - DNA, 50 bp, synthetic construct
  misc_feature 1..50: note = Description of Artificial Sequence: Synthetic oligonucleotide
  source 1..50: mol_type = other DNA
tacagaatactgccgccagctggatttcccaattctgagtaacactctgc

SEQ ID NO: 214 - DNA, 50 bp, synthetic construct
  misc_feature 1..50: note = Description of Artificial Sequence: Synthetic oligonucleotide
  source 1..50: mol_type = other DNA
gaaaagttttacaaaccgagcggtgtctgtgagactttcattcacaccca

SEQ ID NO: 215 - DNA, 20 bp, synthetic construct
  misc_feature 1..20: note = Description of Artificial Sequence: Synthetic oligonucleotide
  source 1..20: mol_type = other DNA
ataatttctattatattaca

SEQ ID NO: 216 - DNA, 20 bp, synthetic construct
  misc_feature 1..20: note = Description of Artificial Sequence: Synthetic oligonucleotide
  source 1..20: mol_type = other DNA
atttcaggtaagccgaggtt

SEQ ID NO: 217 - DNA, 20 bp, synthetic construct
  misc_feature 1..20: note = Description of Artificial Sequence: Synthetic oligonucleotide
  source 1..20: mol_type = other DNA
atactgccgccagctggatt

SEQ ID NO: 218 - DNA, 60 bp, synthetic construct
  misc_feature 1..60: note = Description of Artificial Sequence: Synthetic oligonucleotide
  source 1..60: mol_type = other DNA
tgccgccagctggatttcccaattctgagtaacactctgcaatccaaacagggttcaacc

SEQ ID NO: 219 - DNA, 60 bp, synthetic construct
  misc_feature 1..60: note = Description of Artificial Sequence: Synthetic oligonucleotide
  source 1..60: mol_type = other DNA
tcttgtgtctactgtacagaatactgccgccagctggatttcccaattctgagtaacact

SEQ ID NO: 220 - DNA, 100 bp, synthetic construct
  misc_feature 1..100: note = Description of Artificial Sequence: Synthetic polynucleotide
  source 1..100: mol_type = other DNA
tgccgccagctggatttcccaattctgagtaacactctgcaatccaaacagggttcaaccctccaccttacaggcctgcattacaggacttaaacacata

SEQ ID NO: 221 - DNA, 100 bp, synthetic construct
  misc_feature 1..100: note = Description of Artificial Sequence: Synthetic polynucleotide
  source 1..100: mol_type = other DNA
tgataaaaggcgtacataattcttgtgtctactgtacagaatactgccgccagctggatttcccaattctgagtaacactctgcaatccaaacagggttc

SEQ ID NO: 222 - DNA, 100 bp, synthetic construct
  misc_feature 1..100: note = Description of Artificial Sequence: Synthetic polynucleotide
  source 1..100: mol_type = other DNA
tgaattagctgtatcgtcaaggcactcttgcctacgccaccagctccaaccaccacaagtttatattcagtcattttcagcaggcctctctcccgcacct

SEQ ID NO: 223 - DNA, 100 bp, synthetic construct
  misc_feature 1..100: note = Description of Artificial Sequence: Synthetic polynucleotide
  source 1..100: mol_type = other DNA
atcaaaaaaataaactctaccaagggtgacggaagtctctacagcaaggccaagggctcgccagacggcgaacatcaggggtgcatggtgggcactgccc

SEQ ID NO: 224 - DNA, 29 bp, synthetic construct
  misc_feature 1..29: note = Description of Artificial Sequence: Synthetic primer
  source 1..29: mol_type = other DNA
ctctctgtaccttatcttagtgttactga

SEQ ID NO: 225 - DNA, 24 bp, synthetic construct
  misc_feature 1..24: note = Description of Artificial Sequence: Synthetic primer
  source 1..24: mol_type = other DNA
atttctggcatatttctgaaggtg

SEQ ID NO: 226 - DNA, 22 bp, synthetic construct
  misc_feature 1..22: note = Description of Artificial Sequence: Synthetic primer
  source 1..22: mol_type = other DNA
acccttcctttcttaccacaca

SEQ ID NO: 227 - DNA, 23 bp, synthetic construct
  misc_feature 1..23: note = Description of Artificial Sequence: Synthetic primer
  source 1..23: mol_type = other DNA
cagggtgtccagatctgattgtt

SEQ ID NO: 228 - DNA, 29 bp, synthetic construct
  misc_feature 1..29: note = Description of Artificial Sequence: Synthetic primer
  source 1..29: mol_type = other DNA
cttctcttttaaactaacccatcagagtt

SEQ ID NO: 229 - DNA, 27 bp, synthetic construct
  misc_feature 1..27: note = Description of Artificial Sequence: Synthetic primer
  source 1..27: mol_type = other DNA
caagcagtcagaccaaaatacctactg

SEQ ID NO: 230 - DNA, 25 bp, synthetic construct
  misc_feature 1..25: note = Description of Artificial Sequence: Synthetic primer
  source 1..25: mol_type = other DNA
tcttagcatgcttcgatgtggcata

SEQ ID NO: 231 - DNA, 20 bp, synthetic construct
  misc_feature 1..20: note = Description of Artificial Sequence: Synthetic primer
  source 1..20: mol_type = other DNA
catcaacaagccagggcctg

SEQ ID NO: 232 - DNA, 23 bp, synthetic construct
  misc_feature 1..23: note = Description of Artificial Sequence: Synthetic primer
  source 1..23: mol_type = other DNA
gaagaggaaatgtccgtctccac

SEQ ID NO: 233 - DNA, 19 bp, synthetic construct
  misc_feature 1..19: note = Description of Artificial Sequence: Synthetic primer
  source 1..19: mol_type = other DNA
aggcctgtaaggtggaggg

SEQ ID NO: 234 - DNA, 32 bp, synthetic construct
  misc_feature 1..32: note = Description of Artificial Sequence: Synthetic primer
  source 1..32: mol_type = other DNA
tgaaataacggcaatttatccattgcacatac

SEQ ID NO: 235 - DNA, 19 bp, synthetic construct
  misc_feature 1..19: note = Description of Artificial Sequence: Synthetic primer
  source 1..19: mol_type = other DNA
gggagcagcatggagcctt

SEQ ID NO: 236 - DNA, 22 bp, synthetic construct
  misc_feature 1..22: note = Description of Artificial Sequence: Synthetic primer
  source 1..22: mol_type = other DNA
tccgaccgtaactattcggtgc

SEQ ID NO: 237 - DNA, 23 bp, synthetic construct
  misc_feature 1..23: note = Description of Artificial Sequence: Synthetic primer
  source 1..23: mol_type = other DNA
tgggtgtgaaccatgagaagtat

SEQ ID NO: 238 - DNA, 20 bp, synthetic construct
  misc_feature 1..20: note = Description of Artificial Sequence: Synthetic primer
  source 1..20: mol_type = other DNA
tggcatggactgtggtcatg

SEQ ID NO: 239 - DNA, 23 bp, synthetic construct
  misc_feature 1..23: note = Description of Artificial Sequence: Synthetic primer
  source 1..23: mol_type = other DNA
cctaacttattgcctgggcagtg

SEQ ID NO: 240 - DNA, 25 bp, synthetic construct
  misc_feature 1..25: note = Description of Artificial Sequence: Synthetic primer
  source 1..25: mol_type = other DNA
gcatcagcagtatcttagccatcaa

SEQ ID NO: 241 - DNA, 18 bp, synthetic construct
  misc_feature 1..18: note = Description of Artificial Sequence: Synthetic primer
  source 1..18: mol_type = other DNA
cagaggctcagcggctcc

SEQ ID NO: 242 - DNA, 22 bp, synthetic construct
  misc_feature 1..22: note = Description of Artificial Sequence: Synthetic primer
  source 1..22: mol_type = other DNA
tagctgtatcgtcaaggcactc

SEQ ID NO: 243 - DNA, 22 bp, synthetic construct
  misc_feature 1..22: note = Description of Artificial Sequence: Synthetic primer
  source 1..22: mol_type = other DNA
cacacctgtctgtgcacttgta

SEQ ID NO: 244 - DNA, 20 bp, synthetic construct
  misc_feature 1..20: note = Description of Artificial Sequence: Synthetic primer
  source 1..20: mol_type = other DNA
cggtccacagctcaggaacc

SEQ ID NO: 245 - DNA, 20 bp, synthetic construct
  misc_feature 1..20: note = Description of Artificial Sequence: Synthetic primer
  source 1..20: mol_type = other DNA
accagaaggcggatgatggg

SEQ ID NO: 246 - DNA, 20 bp, synthetic construct
  misc_feature 1..20: note = Description of Artificial Sequence: Synthetic primer
  source 1..20: mol_type = other DNA
ctcagacagcccatccaacc

SEQ ID NO: 247 - DNA, 27 bp, synthetic construct
  misc_feature 1..27: note = Description of Artificial Sequence: Synthetic primer
  source 1..27: mol_type = other DNA
tactacttgcttcctgtaggaatcctc

SEQ ID NO: 248 - DNA, 21 bp, synthetic construct
  misc_feature 1..21: note = Description of Artificial Sequence: Synthetic primer
  source 1..21: mol_type = other DNA
agccctgctgcttcctaactt

SEQ ID NO: 249 - DNA, 26 bp, synthetic construct
  misc_feature 1..26: note = Description of Artificial Sequence: Synthetic primer
  source 1..26: mol_type = other DNA
accctagtttatttcagcatcagcag

SEQ ID NO: 250 - skipped

SEQ ID NO: 251 - DNA, 190 bp, synthetic construct
  misc_feature 1..190: note = Description of Artificial Sequence: Synthetic polynucleotide
  modified_base 46..95: mod_base = OTHER; note = a, c, t, g, unknown or other
  modified_base 97..145: mod_base = OTHER; note = a, c, t, g, unknown or other
  source 1..190: mol_type = other DNA
gtggaatagtataacaatatgctaaatgttgttatagtatcccacnnnnnnnnnnnnnnnnnnnnnnnnnnnnnnnnnnnnnnnnnnnnnnnnnncnnnnnnnnnnnnnnnnnnnnnnnnnnnnnnnnnnnnnnnnnnnnnnnnngtggaatagtataacaatatgctaaatgttgttatagtatcccac

SEQ ID NO: 252 - DNA, 46 bp, unidentified
  misc_feature 1..46: note = Description of Unknown: target sequence
  source 1..46: mol_type = other DNA
tgaatgaaagtctcacagacaccgctcagtttgtaaaacttttctt

SEQ ID NO: 253 - DNA, 24 bp, unidentified
  misc_feature 1..24: note = Description of Unknown: target sequence
  source 1..24: mol_type = other DNA
tcacagacaccgctcagtttgtaa

SEQ ID NO: 254 - DNA, 25 bp, synthetic construct
  misc_feature 1..25: note = Description of Artificial Sequence: Synthetic oligonucleotide
  source 1..25: mol_type = other DNA
cagacaccgctcagtttgtaaaact

SEQ ID NO: 255 - DNA, 25 bp, synthetic construct
  misc_feature 1..25: note = Description of Artificial Sequence: Synthetic oligonucleotide
  source 1..25: mol_type = other DNA
ggaaatccagctagcggcagtattc